European Patent Specification EP 3 532 626 B1, published August 30, 2023. Title: METHOD FOR PRODUCING OBJECTIVE SUBSTANCE. Applicant: Ajinomoto Co., Inc. The sequence listing filed with the application follows.

SEQUENCE LISTING (187 sequences)

SEQ ID NO: 1 - DNA, 1053 bp, Escherichia coli
atgaattatcagaacgacgatttacgcatcaaagaaatcaaagagttacttcctcctgtcgcattgctggaaaaattccccgctactgaaaatgccgcgaatacggttgcccatgcccgaaaagcgatccataagatcctgaaaggtaatgatgatcgcctgttggttgtgattggcccatgctcaattcatgatcctgtcgcggcaaaagagtatgccactcgcttgctggcgctgcgtgaagagctgaaagatgagctggaaatcgtaatgcgcgtctattttgaaaagccgcgtaccacggtgggctggaaagggctgattaacgatccgcatatggataatagcttccagatcaacgacggtctgcgtatagcccgtaaattgctgcttgatattaacgacagcggtctgccagcggcaggtgagtttctcgatatgatcaccccacaatatctcgctgacctgatgagctggggcgcaattggcgcacgtaccaccgaatcgcaggtgcaccgcgaactggcatcagggctttcttgtccggtcggcttcaaaaatggcaccgacggtacgattaaagtggctatcgatgccattaatgccgccggtgcgccgcactgcttcctgtccgtaacgaaatgggggcattcggcgattgtgaataccagcggtaacggcgattgccatatcattctgcgcggcggtaaagagcctaactacagcgcgaagcacgttgctgaagtgaaagaagggctgaacaaagcaggcctgccagcacaggtgatgatcgatttcagccatgctaactcgtccaaacaattcaaaaagcagatggatgtttgtgctgacgtttgccagcagattgccggtggcgaaaaggccattattggcgtgatggtggaaagccatctggtggaaggcaatcagagcctcgagagcggggagccgctggcctacggtaagagcatcaccgatgcctgcatcggctgggaagataccgatgctctgttacgtcaactggcgaatgcagtaaaagcgcgtcgcgggtaa

SEQ ID NO: 2 - protein, 350 aa, Escherichia coli
MNYQNDDLRIKEIKELLPPVALLEKFPATENAANTVAHARKAIHKILKGNDDRLLVVIGPCSIHDPVAAKEYATRLLALREELKDELEIVMRVYFEKPRTTVGWKGLINDPHMDNSFQINDGLRIARKLLLDINDSGLPAAGEFLDMITPQYLADLMSWGAIGARTTESQVHRELASGLSCPVGFKNGTDGTIKVAIDAINAAGAPHCFLSVTKWGHSAIVNTSGNGDCHIILRGGKEPNYSAKHVAEVKEGLNKAGLPAQVMIDFSHANSSKQFKKQMDVCADVCQQIAGGEKAIIGVMVESHLVEGNQSLESGEPLAYGKSITDACIGWEDTDALLRQLANAVKARRG

SEQ ID NO: 3 - DNA, 1089 bp, Escherichia coli
atggagaggattgtcgttactctcggggaacgtagttacccaattaccatcgcatctggtttgtttaatgaaccagcttcattcttaccgctgaaatcgggcgagcaggtcatgttggtcaccaacgaaaccctggctcctctgtatctcgataaggtccgcggcgtacttgaacaggcgggtgttaacgtcgatagcgttatcctccctgacggcgagcagtataaaagcctggctgtactcgataccgtctttacggcgttgttacaaaaaccgcatggtcgcgatactacgctggtggcgcttggcggcggcgtagtgggcgatctgaccggcttcgcggcggcgagttatcagcgcggtgtccgtttcattcaagtcccgacgacgttactgtcgcaggtcgattcctccgttggcggcaaaactgcggtcaaccatcccctcggtaaaaacatgattggcgcgttctaccaacctgcttcagtggtggtggatctcgactgtctgaaaacgcttcccccgcgtgagttagcgtcggggctggcagaagtcatcaaatacggcattattcttgacggtgcgttttttaactggctggaagagaatctggatgcgttgttgcgtctggacggtccggcaatggcgtactgtattcgccgttgttgtgaactgaaggcagaagttgtcgccgccgacgagcgcgaaaccgggttacgtgctttactgaatctgggacacacctttggtcatgccattgaagctgaaatggggtatggcaattggttacatggtgaagcggtcgctgcgggtatggtgatggcggcgcggacgtcggaacgtctcgggcagtttagttctgccgaaacgcagcgtattataaccctgctcaagcgggctgggttaccggtcaatgggccgcgcgaaatgtccgcgcaggcgtatttaccgcatatgctgcgtgacaagaaagtccttgcgggagagatgcgcttaattcttccgttggcaattggtaagagtgaagttcgcagcggcgtttcgcacgagcttgttcttaacgccattgccgattgtcaatcagcgtaa

SEQ ID NO: 4 - protein, 362 aa, Escherichia coli
MERIVVTLGERSYPITIASGLFNEPASFLPLKSGEQVMLVTNETLAPLYLDKVRGVLEQAGVNVDSVILPDGEQYKSLAVLDTVFTALLQKPHGRDTTLVALGGGVVGDLTGFAAASYQRGVRFIQVPTTLLSQVDSSVGGKTAVNHPLGKNMIGAFYQPASVVVDLDCLKTLPPRELASGLAEVIKYGIILDGAFFNWLEENLDALLRLDGPAMAYCIRRCCELKAEVVAADERETGLRALLNLGHTFGHAIEAEMGYGNWLHGEAVAAGMVMAARTSERLGQFSSAETQRIITLLKRAGLPVNGPREMSAQAYLPHMLRDKKVLAGEMRLILPLAIGKSEVRSGVSHELVLNAIADCQSA

SEQ ID NO: 5 - DNA, 759 bp, Escherichia coli
atgaaaaccgtaactgtaaaagatctcgtcattggtacgggcgcacctaaaatcatcgtctcgctgatggcgaaagatatcgccagcgtgaaatccgaagctctcgcctatcgtgaagcggactttgatattctggaatggcgtgtggaccactatgccgacctctccaatgtggagtctgtcatggcggcagcaaaaattctccgtgagaccatgccagaaaaaccgctgctgtttaccttccgcagtgccaaagaaggcggcgagcaggcgatttccaccgaggcttatattgcactcaatcgtgcagccatcgacagcggcctggttgatatgatcgatctggagttatttaccggtgatgatcaggttaaagaaaccgtcgcctacgcccacgcgcatgatgtgaaagtagtcatgtccaaccatgacttccataaaacgccggaagccgaagaaatcattgcccgtctgcgcaaaatgcaatccttcgacgccgatattcctaagattgcgctgatgccgcaaagtaccagcgatgtgctgacgttgcttgccgcgaccctggagatgcaggagcagtatgccgatcgtccaattatcacgatgtcgatggcaaaaactggcgtaatttctcgtctggctggtgaagtatttggctcggcggcaacttttggtgcggtaaaaaaagcgtctgcgccagggcaaatctcggtaaatgatttgcgcacggtattaactattttacaccaggcataa

SEQ ID NO: 6 - protein, 252 aa, Escherichia coli
MKTVTVKDLVIGTGAPKIIVSLMAKDIASVKSEALAYREADFDILEWRVDHYADLSNVESVMAAAKILRETMPEKPLLFTFRSAKEGGEQAISTEAYIALNRAAIDSGLVDMIDLELFTGDDQVKETVAYAHAHDVKVVMSNHDFHKTPEAEEIIARLRKMQSFDADIPKIALMPQSTSDVLTLLAATLEMQEQYADRPIITMSMAKTGVISRLAGEVFGSAATFGAVKKASAPGQISVNDLRTVLTILHQA

SEQ ID NO: 7 - DNA, 843 bp, Bacillus thuringiensis
atgaaatattcgctatgtaccatttcatttcgtcatcaattaatttcatttactgatattgttcaatttgcatatgaaaacggttttgaaggaattgaattatgggggacgcatgcacaaaatttgtacatgcaagaacgtgaaacgacagaacgagaattgaattttctaaaggataaaaacttagaaattacgatgataagtgattacttagatatatcattatcagcagattttgaaaaaacgatagagaaaagtgaacaacttgtagtactagctaattggtttaatacgaataaaattcgcacgtttgctgggcaaaaagggagcaaggacttctcggaacaagagagaaaagagtatgtgaagcgaatacgtaagatttgtgatgtgtttgctcagaacaatatgtatgtgctgttagaaacacatcccaatacactaacggacacattgccttctactatagagttattagaagaagtaaaccatccgaatttaaaaataaatcttgattttcttcatatatgggagtctggcgcagatccaatagacagtttccatcgattaaagccgtggacactacattaccattttaagaatatatcttcagcggattatttgcatgtgtttgaacctaataatgtatatgctgcagcaggaagtcgtataggtatggttccgttatttgaaggtattgtaaattatgatgagattattcaggaagtgagaaatacggatctttttgcttccttagaatggtttggacataattcaaaagagatattaaaagaagaaatgaaagtattaataaatagaaaattagaagtagtaacttcgtaa

SEQ ID NO: 8 - protein, 280 aa, Bacillus thuringiensis
MKYSLCTISFRHQLISFTDIVQFAYENGFEGIELWGTHAQNLYMQERETTERELNFLKDKNLEITMISDYLDISLSADFEKTIEKSEQLVVLANWFNTNKIRTFAGQKGSKDFSEQERKEYVKRIRKICDVFAQNNMYVLLETHPNTLTDTLPSTIELLEEVNHPNLKINLDFLHIWESGADPIDSFHRLKPWTLHYHFKNISSADYLHVFEPNNVYAAAGSRIGMVPLFEGIVNYDEIIQEVRNTDLFASLEWFGHNSKEILKEEMKVLINRKLEVVTS

SEQ ID NO: 9 - DNA, 1542 bp, Escherichia coli
atgcgtctggaagtcttttgtgaagaccgactcggtctgacccgcgaattactcgatctactcgtgctaagaggcattgatttacgcggtattgagattgatcccattgggcgaatctacctcaattttgctgaactggagtttgagagtttcagcagtctgatggccgaaatacgccgtattgcgggtgttaccgatgtgcgtactgtcccgtggatgccttccgaacgtgagcatctggcgttgagcgcgttactggaggcgttgcctgaacctgtgctctctgtcgatatgaaaagcaaagtggatatggcgaacccggcgagctgtcagctttttgggcaaaaattggatcgcctgcgcaaccataccgccgcacaattgattaacggctttaattttttacgttggctggaaagcgaaccgcaagattcgcataacgagcatgtcgttattaatgggcagaatttcctgatggagattacgcctgtttatcttcaggatgaaaatgatcaacacgtcctgaccggtgcggtggtgatgttgcgatcaacgattcgtatgggccgccagttgcaaaatgtcgccgcccaggacgtcagcgccttcagtcaaattgtcgccgtcagcccgaaaatgaagcatgttgtcgaacaggcgcagaaactggcgatgctaagcgcgccgctgctgattacgggtgacacaggtacaggtaaagatctctttgcctacgcctgccatcaggcaagccccagagcgggcaaaccttacctggcgctgaactgtgcgtctataccggaagatgcggtcgagagtgaactgtttggtcatgctccggaagggaagaaaggattctttgagcaggcgaacggtggttcggtgctgttggatgaaataggggaaatgtcaccacggatgcaggcgaaattactgcgtttccttaatgatggcactttccgtcgggttggcgaagaccatgaggtgcatgtcgatgtgcgggtgatttgcgctacgcagaagaatctggtcgaactggtgcaaaaaggcatgttccgtgaagatctctattatcgtctgaacgtgttgacgctcaatctgccgccgctacgtgactgtccgcaggacatcatgccgttaactgagctgttcgtcgcccgctttgccgacgagcagggcgtgccgcgtccgaaactggccgctgacctgaatactgtacttacgcgttatgcgtggccgggaaatgtgcggcagttaaagaacgctatctatcgcgcactgacacaactggacggttatgagctgcgtccacaggatattttgttgccggattatgacgccgcaacggtagccgtgggcgaagatgcgatggaaggttcgctggacgaaatcaccagccgttttgaacgctcggtattaacccagctttatcgcaattatcccagcacgcgcaaactggcaaaacgtctcggcgtttcacataccgcgattgccaataagttgcgggaatatggtctgagtcagaagaagaacgaagagtaa

SEQ ID NO: 10 - protein, 513 aa, Escherichia coli
MRLEVFCEDRLGLTRELLDLLVLRGIDLRGIEIDPIGRIYLNFAELEFESFSSLMAEIRRIAGVTDVRTVPWMPSEREHLALSALLEALPEPVLSVDMKSKVDMANPASCQLFGQKLDRLRNHTAAQLINGFNFLRWLESEPQDSHNEHVVINGQNFLMEITPVYLQDENDQHVLTGAVVMLRSTIRMGRQLQNVAAQDVSAFSQIVAVSPKMKHVVEQAQKLAMLSAPLLITGDTGTGKDLFAYACHQASPRAGKPYLALNCASIPEDAVESELFGHAPEGKKGFFEQANGGSVLLDEIGEMSPRMQAKLLRFLNDGTFRRVGEDHEVHVDVRVICATQKNLVELVQKGMFREDLYYRLNVLTLNLPPLRDCPQDIMPLTELFVARFADEQGVPRPKLAADLNTVLTRYAWPGNVRQLKNAIYRALTQLDGYELRPQDILLPDYDAATVAVGEDAMEGSLDEITSRFERSVLTQLYRNYPSTRKLAKRLGVSHTAIANKLREYGLSQKKNEE

SEQ ID NO: 11 - DNA, 2304 bp, Homo sapiens
cggcctgcgtccgccaccggaagcgccctcctaatccccgcagcgccaccgccattgccgccatcgtcgtggggcttctggggcagctagggctgcccgccgcgctgcctgcgccggaccggggcgggtccagtcccgggcgggccgtcgcgggagagaaataacatctgctttgctgccgagctcagaggagaccccagacccctcccgcagccagagggctggagcctgctcagaggtgctttgaagatgccggaggccccgcctctgctgttggcagctgtgttgctgggcctggtgctgctggtggtgctgctgctgcttctgaggcactggggctggggcctgtgccttatcggctggaacgagttcatcctgcagcccatccacaacctgctcatgggtgacaccaaggagcagcgcatcctgaaccacgtgctgcagcatgcggagcccgggaacgcacagagcgtgctggaggccattgacacctactgcgagcagaaggagtgggccatgaacgtgggcgacaagaaaggcaagatcgtggacgccgtgattcaggagcaccagccctccgtgctgctggagctgggggcctactgtggctactcagctgtgcgcatggcccgcctgctgtcaccaggggcgaggctcatcaccatcgagatcaaccccgactgtgccgccatcacccagcggatggtggatttcgctggcgtgaaggacaaggtcacccttgtggttggagcgtcccaggacatcatcccccagctgaagaagaagtatgatgtggacacactggacatggtcttcctcgaccactggaaggaccggtacctgccggacacgcttctcttggaggaatgtggcctgctgcggaaggggacagtgctactggctgacaacgtgatctgcccaggtgcgccagacttcctagcacacgtgcgcgggagcagctgctttgagtgcacacactaccaatcgttcctggaatacagggaggtggtggacggcctggagaaggccatctacaagggcccaggcagcgaagcagggccctgactgcccccccggcccccctctcgggctctctcacccagcctggtactgaaggtgccagacgtgctcctgctgaccttctgcggctccgggctgtgtcctaaatgcaaagcacacctcggccgaggcctgcgccctgacatgctaacctctctgaactgcaacactggattgttcttttttaagactcaatcatgacttctttactaacactggctagctatattatcttatatactaatatcatgttttaaaaatataaaatagaaattaagaatctaaatatttagatataactcgacttagtacatccttctcaactgccattcccctgctgcccttgacttgggcaccaaacattcaaagctccccttgacggacgctaacgctaagggcggggcccctagctggctgggttctgggtggcacgcctggcccactggcctcccagccacagtggtgcagaggtcagccctcctgcagctaggccaggggcacctgttagccccatggggacgactgccggcctgggaaacgaagaggagtcagccagcattcacacctttctgaccaagcaggcgctggggacaggtggaccccgcagcagcaccagcccctctgggccccatgtggcacagagtggaagcatctccttccctactccccactgggccttgcttacagaagaggcaatggctcagaccagctcccgcatccctgtagttgcctccctggcccatgagtgaggatgcagtgctggtttctgcccacctacacctagagctgtccccatctcctccaaggggtcagactgctagccacctcagaggctccaagggcccagttcccaggcccaggacaggaatcaaccctgtgctagctgagttcacctgcaccgagaccagcccctagccaagattctactcctgggctcaaggcctggctagcccccagccagcccactcctatggatagacagaccagtgagcccaagtggacaagtttggggccacccagggaccagaaacagagcctctgcaggacacagcagatgggcacctgggaccacctccacccagggccctgccccagacgcgcagaggcccgacacaagggagaagccagccacttgtgccagacctgagtggcagaaagcaaaaagttcctttgctgctttaatttttaaattttcttacaaaaatttaggtgtttaccaatagtcttattttggcttatttttaa

SEQ ID NO: 12 - DNA, 2262 bp, Homo sapiens
ctcccacgggaggagcaagaacacagaacagagggggcaagacagctccaccaggagtcaggagtgaatcccctctgggaacgaggcactaggaagaagaacttccagcccaggagaaataacatctgctttgctgccgagctcagaggagaccccagacccctcccgcagccagagggctggagcctgctcagaggtgctttgaagatgccggaggccccgcctctgctgttggcagctgtgttgctgggcctggtgctgctggtggtgctgctgctgcttctgaggcactggggctggggcctgtgccttatcggctggaacgagttcatcctgcagcccatccacaacctgctcatgggtgacaccaaggagcagcgcatcctgaaccacgtgctgcagcatgcggagcccgggaacgcacagagcgtgctggaggccattgacacctactgcgagcagaaggagtgggccatgaacgtgggcgacaagaaaggcaagatcgtggacgccgtgattcaggagcaccagccctccgtgctgctggagctgggggcctactgtggctactcagctgtgcgcatggcccgcctgctgtcaccaggggcgaggctcatcaccatcgagatcaaccccgactgtgccgccatcacccagcggatggtggatttcgctggcgtgaaggacaaggtcacccttgtggttggagcgtcccaggacatcatcccccagctgaagaagaagtatgatgtggacacactggacatggtcttcctcgaccactggaaggaccggtacctgccggacacgcttctcttggaggaatgtggcctgctgcggaaggggacagtgctactggctgacaacgtgatctgcccaggtgcgccagacttcctagcacacgtgcgcgggagcagctgctttgagtgcacacactaccaatcgttcctggaatacagggaggtggtggacggcctggagaaggccatctacaagggcccaggcagcgaagcagggccctgactgcccccccggcccccctctcgggctctctcacccagcctggtactgaaggtgccagacgtgctcctgctgaccttctgcggctccgggctgtgtcctaaatgcaaagcacacctcggccgaggcctgcgccctgacatgctaacctctctgaactgcaacactggattgttcttttttaagactcaatcatgacttctttactaacactggctagctatattatcttatatactaatatcatgttttaaaaatataaaatagaaattaagaatctaaatatttagatataactcgacttagtacatccttctcaactgccattcccctgctgcccttgacttgggcaccaaacattcaaagctccccttgacggacgctaacgctaagggcggggcccctagctggctgggttctgggtggcacgcctggcccactggcctcccagccacagtggtgcagaggtcagccctcctgcagctaggccaggggcacctgttagccccatggggacgactgccggcctgggaaacgaagaggagtcagccagcattcacacctttctgaccaagcaggcgctggggacaggtggaccccgcagcagcaccagcccctctgggccccatgtggcacagagtggaagcatctccttccctactccccactgggccttgcttacagaagaggcaatggctcagaccagctcccgcatccctgtagttgcctccctggcccatgagtgaggatgcagtgctggtttctgcccacctacacctagagctgtccccatctcctccaaggggtcagactgctagccacctcagaggctccaagggcccagttcccaggcccaggacaggaatcaaccctgtgctagctgagttcacctgcaccgagaccagcccctagccaagattctactcctgggctcaaggcctggctagcccccagccagcccactcctatggatagacagaccagtgagcccaagtggacaagtttggggccacccagggaccagaaacagagcctctgcaggacacagcagatgggcacctgggaccacctccacccagggccctgccccagacgcgcagaggcccgacacaagggagaagccagccacttgtgccagacctgagtggcagaaagcaaaaagttcctttgctgctttaatttttaaattttcttacaaaaatttaggtgtttaccaatagtcttattttggcttatttttaa

SEQ ID NO: 13 - DNA, 2279 bp, Homo sapiens
tggagataacacggatcgctgtgtacactgtgtgctccggttgttgcatccgagggttgatcggatggtggttcccatccagatccaagtcctggcccctgatcacagagaaacacagctggacattaaagtgaaataacatctgctttgctgccgagctcagaggagaccccagacccctcccgcagccagagggctggagcctgctcagaggtgctttgaagatgccggaggccccgcctctgctgttggcagctgtgttgctgggcctggtgctgctggtggtgctgctgctgcttctgaggcactggggctggggcctgtgccttatcggctggaacgagttcatcctgcagcccatccacaacctgctcatgggtgacaccaaggagcagcgcatcctgaaccacgtgctgcagcatgcggagcccgggaacgcacagagcgtgctggaggccattgacacctactgcgagcagaaggagtgggccatgaacgtgggcgacaagaaaggcaagatcgtggacgccgtgattcaggagcaccagccctccgtgctgctggagctgggggcctactgtggctactcagctgtgcgcatggcccgcctgctgtcaccaggggcgaggctcatcaccatcgagatcaaccccgactgtgccgccatcacccagcggatggtggatttcgctggcgtgaaggacaaggtcacccttgtggttggagcgtcccaggacatcatcccccagctgaagaagaagtatgatgtggacacactggacatggtcttcctcgaccactggaaggaccggtacctgccggacacgcttctcttggaggaatgtggcctgctgcggaaggggacagtgctactggctgacaacgtgatctgcccaggtgcgccagacttcctagcacacgtgcgcgggagcagctgctttgagtgcacacactaccaatcgttcctggaatacagggaggtggtggacggcctggagaaggccatctacaagggcccaggcagcgaagcagggccctgactgcccccccggcccccctctcgggctctctcacccagcctggtactgaaggtgccagacgtgctcctgctgaccttctgcggctccgggctgtgtcctaaatgcaaagcacacctcggccgaggcctgcgccctgacatgctaacctctctgaactgcaacactggattgttcttttttaagactcaatcatgacttctttactaacactggctagctatattatcttatatactaatatcatgttttaaaaatataaaatagaaattaagaatctaaatatttagatataactcgacttagtacatccttctcaactgccattcccctgctgcccttgacttgggcaccaaacattcaaagctccccttgacggacgctaacgctaagggcggggcccctagctggctgggttctgggtggcacgcctggcccactggcctcccagccacagtggtgcagaggtcagccctcctgcagctaggccaggggcacctgttagccccatggggacgactgccggcctgggaaacgaagaggagtcagccagcattcacacctttctgaccaagcaggcgctggggacaggtggaccccgcagcagcaccagcccctctgggccccatgtggcacagagtggaagcatctccttccctactccccactgggccttgcttacagaagaggcaatggctcagaccagctcccgcatccctgtagttgcctccctggcccatgagtgaggatgcagtgctggtttctgcccacctacacctagagctgtccccatctcctccaaggggtcagactgctagccacctcagaggctccaagggcccagttcccaggcccaggacaggaatcaaccctgtgctagctgagttcacctgcaccgagaccagcccctagccaagattctactcctgggctcaaggcctggctagcccccagccagcccactcctatggatagacagaccagtgagcccaagtggacaagtttggggccacccagggaccagaaacagagcctctgcaggacacagcagatgggcacctgggaccacctccacccagggccctgccccagacgcgcagaggcccgacacaagggagaagccagccacttgtgccagacctgagtggcagaaagcaaaaagttcctttgctgctttaatttttaaattttcttacaaaaatttaggtgtttaccaatagtcttattttggcttatttttaa

SEQ ID NO: 14 - DNA, 2035 bp, Homo sapiens
gctgttggcagctgtgttgctgggcctggtgctgctggtggtgctgctgctgcttctgaggcactggggctggggcctgtgccttatcggctggaacgagttcatcctgcagcccatccacaacctgctcatgggtgacaccaaggagcagcgcatcctgaaccacgtgctgcagcatgcggagcccgggaacgcacagagcgtgctggaggccattgacacctactgcgagcagaaggagtgggccatgaacgtgggcgacaagaaaggcaagatcgtggacgccgtgattcaggagcaccagccctccgtgctgctggagctgggggcctactgtggctactcagctgtgcgcatggcccgcctgctgtcaccaggggcgaggctcatcaccatcgagatcaaccccgactgtgccgccatcacccagcggatggtggatttcgctggcgtgaaggacaaggtcacccttgtggttggagcgtcccaggacatcatcccccagctgaagaagaagtatgatgtggacacactggacatggtcttcctcgaccactggaaggaccggtacctgccggacacgcttctcttggaggaatgtggcctgctgcggaaggggacagtgctactggctgacaacgtgatctgcccaggtgcgccagacttcctagcacacgtgcgcgggagcagctgctttgagtgcacacactaccaatcgttcctggaatacagggaggtggtggacggcctggagaaggccatctacaagggcccaggcagcgaagcagggccctgactgcccccccggcccccctctcgggctctctcacccagcctggtactgaaggtgccagacgtgctcctgctgaccttctgcggctccgggctgtgtcctaaatgcaaagcacacctcggccgaggcctgcgccctgacatgctaacctctctgaactgcaacactggattgttcttttttaagactcaatcatgacttctttactaacactggctagctatattatcttatatactaatatcatgttttaaaaatataaaatagaaattaagaatctaaatatttagatataactcgacttagtacatccttctcaactgccattcccctgctgcccttgacttgggcaccaaacattcaaagctccccttgacggacgctaacgctaagggcggggcccctagctggctgggttctgggtggcacgcctggcccactggcctcccagccacagtggtgcagaggtcagccctcctgcagctaggccaggggcacctgttagccccatggggacgactgccggcctgggaaacgaagaggagtcagccagcattcacacctttctgaccaagcaggcgctggggacaggtggaccccgcagcagcaccagcccctctgggccccatgtggcacagagtggaagcatctccttccctactccccactgggccttgcttacagaagaggcaatggctcagaccagctcccgcatccctgtagttgcctccctggcccatgagtgaggatgcagtgctggtttctgcccacctacacctagagctgtccccatctcctccaaggggtcagactgctagccacctcagaggctccaagggcccagttcccaggcccaggacaggaatcaaccctgtgctagctgagttcacctgcaccgagaccagcccctagccaagattctactcctgggctcaaggcctggctagcccccagccagcccactcctatggatagacagaccagtgagcccaagtggacaagtttggggccacccagggaccagaaacagagcctctgcaggacacagcagatgggcacctgggaccacctccacccagggccctgccccagacgcgcagaggcccgacacaagggagaagccagccacttgtgccagacctgagtggcagaaagcaaaaagttcctttgctgctttaatttttaaattttcttacaaaaatttaggtgtttaccaatagtcttattttggcttatttttaa

SEQ ID NO: 15 - protein, 271 aa, Homo sapiens
MPEAPPLLLAAVLLGLVLLVVLLLLLRHWGWGLCLIGWNEFILQPIHNLLMGDTKEQRILNHVLQHAEPGNAQSVLEAIDTYCEQKEWAMNVGDKKGKIVDAVIQEHQPSVLLELGAYCGYSAVRMARLLSPGARLITIEINPDCAAITQRMVDFAGVKDKVTLVVGASQDIIPQLKKKYDVDTLDMVFLDHWKDRYLPDTLLLEECGLLRKGTVLLADNVICPGAPDFLAHVRGSSCFECTHYQSFLEYREVVDGLEKAIYKGPGSEAGP

SEQ ID NO: 16 - protein, 221 aa, Homo sapiens
MGDTKEQRILNHVLQHAEPGNAQSVLEAIDTYCEQKEWAMNVGDKKGKIVDAVIQEHQPSVLLELGAYCGYSAVRMARLLSPGARLITIEINPDCAAITQRMVDFAGVKDKVTLVVGASQDIIPQLKKKYDVDTLDMVFLDHWKDRYLPDTLLLEECGLLRKGTVLLADNVICPGAPDFLAHVRGSSCFECTHYQSFLEYREVVDGLEKAIYKGPGSEAGP

SEQ ID NO: 17 - DNA, 3453 bp, Nocardia brasiliensis
ttgttcgccgaggacgagcaggtgaaagccgcggtgccggaccaggaggtggtcgaggcgatccgggcgcccggcctgcgcctggcacagatcatggccaccgtgatggagcgctatgcggaccgccccgcggtgggacagcgggcgagcgagccggtcaccgagagcggtcgcaccaccttccggctgctcccggaattcgagaccctgacctaccgcgagctgtgggcgcgcgtccgcgcggtggccgccgcgtggcacggagatgccgaaaggcctttgcgggccggggatttcgttgctctgctgggtttcgccggcatcgattacggcaccctcgatctcgcgaacatccatctcggcctcgtcacggtgccgctgcaatccggcgccacggccccgcaactcgccgcgatcctggccgagaccacgccccgggtgctggccgcgacacccgaccatctcgatatcgccgtcgaattgctgaccgggggagcctcgccggaacggctggtggtattcgactaccgccccgcggacgacgatcaccgggcggcgctcgagtccgcgcgcagacggttgagcgacgcgggcagtgcggtggtggtcgagacgctcgacgcggtccgcgcccgcggcagcgaattgccggccgcgccgctgttcgttcccgccgcggacgaggacccgctggctctgctcatctacacctccggcagcaccggcacgcctaagggcgccatgtacaccgaaagactgaaccgcacgacgtggctgagcggggcgaaaggcgtcggcctcacgctcggctacatgccgatgagtcatattgccgggcgggcctcgttcgccggtgtgctggcccgcggcggcacggtctacttcaccgcccgcagcgatatgtcgacgctgttcgaagatctggccctggtgcggccgaccgagatgttcttcgtcccgcgcgtgtgcgacatgatcttccagcgctatcaggccgaactgtcgcggcgcgcgcccgccgcggccgcgagcccggaactcgagcaggaactgaagaccgaactgcgcttgtccgcggtcggggaccgcttactcggggcgatcgcgggcagcgcgccgctgtcggccgagatgcgggagttcatggagtcgctgctggatctggaactgcacgacggctacggctcgaccgaggcgggtatcggcgtactgcaagacaatatcgtccagcgtccgccggtcatcgattacaagctcgtcgacgtgccggaattgggctacttccggacggaccagccgcatccccgcggtgagttgctgttgaaaaccgaagggatgattccgggctacttccggcggcccgaggtgaccgcggagatcttcgacgaggacggtttctacaggaccggtgacatcgtcgccgaactcgaaccggatcggctgatctacctggaccgccgcaacaatgtgctgaaactggcccagggcgagttcgtcacggtcgcccatctggaagcggtgttcgcgaccagtccgctgatccggcagatctacatctacggcaacagcgagcgctcgttcctgctggcggtgatcgtgcccaccgcggacgcgctggccgacggtgtcaccgacgcgctgaacacggcgctgaccgaatccttgcgacagctcgcgaaagaagccgggctgcaatcctatgagctgccgcgcgagttcctggtcgaaaccgaaccgttcaccgtcgagaacggtctgctctccggtatcgcgaaactgttgcggcccaagctcaaggagcactacggcgagcgactcgagcagctgtaccgcgatatcgaggcgaaccgcaacgacgagctgatcgagctgcggcgcaccgcggccgagctgccggtgctcgaaaccgtcacgcgggctgcacgttcgatgctcggactggccgcgtcggagttgcggccggacgcgcatttcaccgatctcggcggtgattcactgtccgcgctgtcgttttcgaccctgctgcaggacatgctcgaggtcgaggtcccggtcggtgtcatcgtgagccccgccaactcgctcgccgatctggcgaaatacatcgaggccgaacggcattcgggggtgcggcggccgagcctgatctcggtgcacggtcccggcaccgagatccgtgccgccgatctcaccctggacaagttcatcgacgagcgcaccctcgctgccgcgaaagcggttccggccgcgccggcccaggcgcagaccgtcctgctcaccggggcgaacggctatctcggccgcttcctgtgcctggaatggctgcagcgactggaccagaccggcggcacgctggtctgcatcgtgcgcggtaccgacgcggccgccgcgcggaagcgcctggatgcggtgttcgacagcggtgatccggagctgctcgaccactaccggaagctggccgccgagcacctcgaggtgctcgcgggcgatatcggcgacccgaatctcggcctggacgaagcgacttggcagcggctcgccgcgaccgtcgacctgatcgtgcaccccgccgccctcgtcaaccatgtgctgccgtacagccagctgttcgggccgaatgtggtcggcaccgccgagatcatccggctggccatcaccgagcgccgtaagcccgtgacgtacctgtcgacggtcgcggtggccgcacaggtcgatcccgccggcttcgacgaggagcgcgatatccgggagatgagcgcggtgcgctccatcgacgccgggtacgcgaacggttacggcaacagcaagtgggccggcgaggtgctgctgcgcgaggcccatgatctgtgcgggctgccggtcgccgtgttccgctcggacatgatcctggcgcacagcaaatacgtcggtcagctcaacgtccccgatgtgttcacccggctcatcctgagcctggcgctcaccggcatcgcaccgtattcgttctacgggacggacagcgccgggcagcgcaggcgggcccactacgacggtctgcccgccgatttcgtcgccgaggcgatcaccaccctcggcgcgcgagccgagtcggggttccatacctacgacgtgtggaacccgtacgacgacggcatctcgctggacgaattcgtcgactggctcggcgatttcggcgtgccgatccagcggatcgacgactacgacgaatggttccggcgtttcgagaccgcgatccgcgcgctgcccgaaaagcagcgcgatgcttcgctgctaccgctgctggacgcacaccggcggccactgcgcgcggtgcgcggttcgctgttgcccgccaagaacttccaggcggcggtgcagtccgcgcggatcggccccgatcaggacatcccgcatctttccccgcagttgatcgacaagtacgtcaccgacctgcgccacctcggcctgctctga

SEQ ID NO: 18 - protein, 1150 aa, Nocardia brasiliensis
MFAEDEQVKAAVPDQEVVEAIRAPGLRLAQIMATVMERYADRPAVGQRASEPVTESGRTTFRLLPEFETLTYRELWARVRAVAAAWHGDAERPLRAGDFVALLGFAGIDYGTLDLANIHLGLVTVPLQSGATAPQLAAILAETTPRVLAATPDHLDIAVELLTGGASPERLVVFDYRPADDDHRAALESARRRLSDAGSAVVVETLDAVRARGSELPAAPLFVPAADEDPLALLIYTSGSTGTPKGAMYTERLNRTTWLSGAKGVGLTLGYMPMSHIAGRASFAGVLARGGTVYFTARSDMSTLFEDLALVRPTEMFFVPRVCDMIFQRYQAELSRRAPAAAASPELEQELKTELRLSAVGDRLLGAIAGSAPLSAEMREFMESLLDLELHDGYGSTEAGIGVLQDNIVQRPPVIDYKLVDVPELGYFRTDQPHPRGELLLKTEGMIPGYFRRPEVTAEIFDEDGFYRTGDIVAELEPDRLIYLDRRNNVLKLAQGEFVTVAHLEAVFATSPLIRQIYIYGNSERSFLLAVIVPTADALADGVTDALNTALTESLRQLAKEAGLQSYELPREFLVETEPFTVENGLLSGIAKLLRPKLKEHYGERLEQLYRDIEANRNDELIELRRTAAELPVLETVTRAARSMLGLAASELRPDAHFTDLGGDSLSALSFSTLLQDMLEVEVPVGVIVSPANSLADLAKYIEAERHSGVRRPSLISVHGPGTEIRAADLTLDKFIDERTLAAAKAVPAAPAQAQTVLLTGANGYLGRFLCLEWLQRLDQTGGTLVCIVRGTDAAAARKRLDAVFDSGDPELLDHYRKLAAEHLEVLAGDIGDPNLGLDEATWQRLAATVDLIVHPAALVNHVLPYSQLFGPNVVGTAEIIRLAITERRKPVTYLSTVAVAAQVDPAGFDEERDIREMSAVRSIDAGYANGYGNSKWAGEVLLREAHDLCGLPVAVFRSDMILAHSKYVGQLNVPDVFTRLILSLALTGIAPYSFYGTDSAGQRRRAHYDGLPADFVAEAITTLGARAESGFHTYDVWNPYDDGISLDEFVDWLGDFGVPIQRIDDYDEWFRRFETAIRALPEKQRDASLLPLLDAHRRPLRAVRGSLLPAKNFQAAVQSARIGPDQDIPHLSPQLIDKYVTDLRHLGLL

SEQ ID NO: 19 - DNA, 3501 bp, Nocardia brasiliensis
atggcgactgattcgcgaagcgatcggctacggcgtcgaattgcacagttgttcgccgaggacgagcaggtgaaagccgcggtgccggaccaggaggtggtcgaggcgatccgggcgcccggcctgcgcctggcacagatcatggccaccgtgatggagcgctatgcggaccgccccgcggtgggacagcgggcgagcgagccggtcaccgagagcggtcgcaccaccttccggctgctcccggaattcgagaccctgacctaccgcgagctgtgggcgcgcgtccgcgcggtggccgccgcgtggcacggagatgccgaaaggcctttgcgggccggggatttcgttgctctgctgggtttcgccggcatcgattacggcaccctcgatctcgcgaacatccatctcggcctcgtcacggtgccgctgcaatccggcgccacggccccgcaactcgccgcgatcctggccgagaccacgccccgggtgctggccgcgacacccgaccatctcgatatcgccgtcgaattgctgaccgggggagcctcgccggaacggctggtggtattcgactaccgccccgcggacgacgatcaccgggcggcgctcgagtccgcgcgcagacggttgagcgacgcgggcagtgcggtggtggtcgagacgctcgacgcggtccgcgcccgcggcagcgaattgccggccgcgccgctgttcgttcccgccgcggacgaggacccgctggctctgctcatctacacctccggcagcaccggcacgcctaagggcgccatgtacaccgaaagactgaaccgcacgacgtggctgagcggggcgaaaggcgtcggcctcacgctcggctacatgccgatgagtcatattgccgggcgggcctcgttcgccggtgtgctggcccgcggcggcacggtctacttcaccgcccgcagcgatatgtcgacgctgttcgaagatctggccctggtgcggccgaccgagatgttcttcgtcccgcgcgtgtgcgacatgatcttccagcgctatcaggccgaactgtcgcggcgcgcgcccgccgcggccgcgagcccggaactcgagcaggaactgaagaccgaactgcgcttgtccgcggtcggggaccgcttactcggggcgatcgcgggcagcgcgccgctgtcggccgagatgcgggagttcatggagtcgctgctggatctggaactgcacgacggctacggctcgaccgaggcgggtatcggcgtactgcaagacaatatcgtccagcgtccgccggtcatcgattacaagctcgtcgacgtgccggaattgggctacttccggacggaccagccgcatccccgcggtgagttgctgttgaaaaccgaagggatgattccgggctacttccggcggcccgaggtgaccgcggagatcttcgacgaggacggtttctacaggaccggtgacatcgtcgccgaactcgaaccggatcggctgatctacctggaccgccgcaacaatgtgctgaaactggcccagggcgagttcgtcacggtcgcccatctggaagcggtgttcgcgaccagtccgctgatccggcagatctacatctacggcaacagcgagcgctcgttcctgctggcggtgatcgtgcccaccgcggacgcgctggccgacggtgtcaccgacgcgctgaacacggcgctgaccgaatccttgcgacagctcgcgaaagaagccgggctgcaatcctatgagctgccgcgcgagttcctggtcgaaaccgaaccgttcaccgtcgagaacggtctgctctccggtatcgcgaaactgttgcggcccaagctcaaggagcactacggcgagcgactcgagcagctgtaccgcgatatcgaggcgaaccgcaacgacgagctgatcgagctgcggcgcaccgcggccgagctgccggtgctcgaaaccgtcacgcgggctgcacgttcgatgctcggactggccgcgtcggagttgcggccggacgcgcatttcaccgatctcggcggtgattcactgtccgcgctgtcgttttcgaccctgctgcaggacatgctcgaggtcgaggtcccggtcggtgtcatcgtgagccccgccaactcgctcgccgatctggcgaaatacatcgaggccgaacggcattcgggggtgcggcggccgagcctgatctcggtgcacggtcccggcaccgagatccgtgccgccgatctcaccctggacaagttcatcgacgagcgcaccctcgctgccgcgaaagcggttccggccgcgccggcccaggcgcagaccgtcctgctcaccggggcgaacggctatctcggccgcttcctgtgcctggaatggctgcagcgactggaccagaccggcggcacgctggtctgcatcgtgcgcggtaccgacgcggccgccgcgcggaagcgcctggatgcggtgttcgacagcggtgatccggagctgctcgaccactaccggaagctggccgccgagcacctcgaggtgctcgcgggcgatatcggcgacccgaatctcggcctggacgaagcgacttggcagcggctcgccgcgaccgtcgacctgatcgtgcaccccgccgccctcgtcaaccatgtgctgccgtacagccagctgttcgggccgaatgtggtcggcaccgccgagatcatccggctggccatcaccgagcgccgtaagcccgtgacgtacctgtcgacggtcgcggtggccgcacaggtcgatcccgccggcttcgacgaggagcgcgatatccgggagatgagcgcggtgcgctccatcgacgccgggtacgcgaacggttacggcaacagcaagtgggccggcgaggtgctgctgcgcgaggcccatgatctgtgcgggctgccggtcgccgtgttccgctcggacatgatcctggcgcacagcaaatacgtcggtcagctcaacgtccccgatgtgttcacccggctcatcctgagcctggcgctcaccggcatcgcaccgtattcgttctacgggacggacagcgccgggcagcgcaggcgggcccactacgacggtctgcccgccgatttcgtcgccgaggcgatcaccaccctcggcgcgcgagccgagtcggggttccatacctacgacgtgtggaacccgtacgacgacggcatctcgctggacgaattcgtcgactggctcggcgatttcggcgtgccgatccagcggatcgacgactacgacgaatggttccggcgtttcgagaccgcgatccgcgcgctgcccgaaaagcagcgcgatgcttcgctgctaccgctgctggacgcacaccggcggccactgcgcgcggtgcgcggttcgctgttgcccgccaagaacttccaggcggcggtgcagtccgcgcggatcggccccgatcaggacatcccgcatctttccccgcagttgatcgacaagtacgtcaccgacctgcgccacctcggcctgctctga

SEQ ID NO: 20 - protein, 1166 aa, Nocardia brasiliensis
MATDSRSDRLRRRIAQLFAEDEQVKAAVPDQEVVEAIRAPGLRLAQIMATVMERYADRPAVGQRASEPVTESGRTTFRLLPEFETLTYRELWARVRAVAAAWHGDAERPLRAGDFVALLGFAGIDYGTLDLANIHLGLVTVPLQSGATAPQLAAILAETTPRVLAATPDHLDIAVELLTGGASPERLVVFDYRPADDDHRAALESARRRLSDAGSAVVVETLDAVRARGSELPAAPLFVPAADEDPLALLIYTSGSTGTPKGAMYTERLNRTTWLSGAKGVGLTLGYMPMSHIAGRASFAGVLARGGTVYFTARSDMSTLFEDLALVRPTEMFFVPRVCDMIFQRYQAELSRRAPAAAASPELEQELKTELRLSAVGDRLLGAIAGSAPLSAEMREFMESLLDLELHDGYGSTEAGIGVLQDNIVQRPPVIDYKLVDVPELGYFRTDQPHPRGELLLKTEGMIPGYFRRPEVTAEIFDEDGFYRTGDIVAELEPDRLIYLDRRNNVLKLAQGEFVTVAHLEAVFATSPLIRQIYIYGNSERSFLLAVIVPTADALADGVTDALNTALTESLRQLAKEAGLQSYELPREFLVETEPFTVENGLLSGIAKLLRPKLKEHYGERLEQLYRDIEANRNDELIELRRTAAELPVLETVTRAARSMLGLAASELRPDAHFTDLGGDSLSALSFSTLLQDMLEVEVPVGVIVSPANSLADLAKYIEAERHSGVRRPSLISVHGPGTEIRAADLTLDKFIDERTLAAAKAVPAAPAQAQTVLLTGANGYLGRFLCLEWLQRLDQTGGTLVCIVRGTDAAAARKRLDAVFDSGDPELLDHYRKLAAEHLEVLAGDIGDPNLGLDEATWQRLAATVDLIVHPAALVNHVLPYSQLFGPNVVGTAEIIRLAITERRKPVTYLSTVAVAAQVDPAGFDEERDIREMSAVRSIDAGYANGYGNSKWAGEVLLREAHDLCGLPVAVFRSDMILAHSKYVGQLNVPDVFTRLILSLALTGIAPYSFYGTDSAGQRRRAHYDGLPADFVAEAITTLGARAESGFHTYDVWNPYDDGISLDEFVDWLGDFGVPIQRIDDYDEWFRRFETAIRALPEKQRDASLLPLLDAHRRPLRAVRGSLLPAKNFQAAVQSARIGPDQDIPHLSPQLIDKYVTDLRHLGLL

SEQ ID NO: 21 - DNA, 621 bp, Escherichia coli
atgaaaactacgcatacctccctcccctttgccggacatacgctgcattttgttgagttcgatccggcgaatttttgtgagcaggatttactctggctgccgcactacgcacaactgcaacacgctggacgtaaacgtaaaacagagcatttagccggacggatcgctgctgtttatgctttgcgggaatatggctataaatgtgtgcccgcaatcggcgagctacgccaacctgtctggcctgcggaggtatacggcagtattagccactgtgggactacggcattagccgtggtatctcgtcaaccgattggcattgatatagaagaaattttttctgtacaaaccgcaagagaattgacagacaacattattacaccagcggaacacgagcgactcgcagactgcggtttagccttttctctggcgctgacactggcattttccgccaaagagagcgcatttaaggcaagtgagatccaaactgatgcaggttttctggactatcagataattagctggaataaacagcaggtcatcattcatcgtgagaatgagatgtttgctgtgcactggcagataaaagaaaagatagtcataacgctgtgccaacacgattaa

SEQ ID NO: 22 - protein, 206 aa, Escherichia coli
MKTTHTSLPFAGHTLHFVEFDPANFCEQDLLWLPHYAQLQHAGRKRKTEHLAGRIAAVYALREYGYKCVPAIGELRQPVWPAEVYGSISHCGTTALAVVSRQPIGIDIEEIFSVQTARELTDNIITPAEHERLADCGLAFSLALTLAFSAKESAFKASEIQTDAGFLDYQIISWNKQQVIIHRENEMFAVHWQIKEKIVITLCQHD

SEQ ID NO: 23 - DNA, 654 bp, Corynebacterium glutamicum
atgctggatgagtctttgtttccaaattcggcaaagttttctttcattaaaactggcgatgctgttaatttagaccatttccatcagttgcatccgttggaaaaggcactggtagcgcactcggttgatattagaaaagcagagtttggagatgccaggtggtgtgcacatcaggcactccaagctttgggacgagatagcggtgatcccattttgcgtggggaacgaggaatgccattgtggccttcttcggtgtctggttcattgacccacactgacggattccgagctgctgttgtggcgccacgattgttggtgcgttctatgggattggatgccgaacctgcggagccgttgcccaaggatgttttgggttcaatcgctcgggtgggggagattcctcaacttaagcgcttggaggaacaaggtgtgcactgcgcggatcgcctgctgttttgtgccaaggaagcaacatacaaagcgtggttcccgctgacgcataggtggcttggttttgaacaagctgagatcgacttgcgtgatgatggcacttttgtgtcctatttgctggttcgaccaactccagtgccgtttatttcaggtaaatgggtactgcgtgatggttatgtcatagctgcgactgcagtgacttga

SEQ ID NO: 24 - protein, 217 aa, Corynebacterium glutamicum
MLDESLFPNSAKFSFIKTGDAVNLDHFHQLHPLEKALVAHSVDIRKAEFGDARWCAHQALQALGRDSGDPILRGERGMPLWPSSVSGSLTHTDGFRAAVVAPRLLVRSMGLDAEPAEPLPKDVLGSIARVGEIPQLKRLEEQGVHCADRLLFCAKEATYKAWFPLTHRWLGFEQAEIDLRDDGTFVSYLLVRPTPVPFISGKWVLRDGYVIAATAVT

SEQ ID NO: 25 - DNA, 1428 bp, Corynebacterium glutamicum
atgcgcctgcgtgtctcgagtagtctcctccccttcctcgtccccaacctcgaccattacggtcgccctctcctaaaggagcctggcatggatatccgccaaacaattaacgacacagcaatgtcgagatatcagtggttcattgtatttatcgcagtgctgctcaacgcactggacggctttgatgtcctcgccatgtcttttactgcgaatgcagtgaccgaagaatttggactgagtggcagccagcttggtgtgctgctgagttccgcgctgttcggcatgaccgctggatctttgctgttcggtccgatcggtgaccgtttcggccgtaagaatgccctgatgatcgcgctgctgttcaacgtggtgggattggtattgtccgccaccgcgcagtccgcaggccagttgggcgtgtggcgtttgatcactggtatcggcatcggcggaatcctcgcctgcatcacagtggtgatcagtgagttctccaacaacaaaaaccgcggcatggccatgtccatctacgctgctggttacggcatcggcgcgtccttgggcggattcggcgcagcgcagctcatcccaacatttggatggcgctccgtgttcgcagccggtgcgatcgcaactggtatcgccaccatcgctactttcttcttcctgccagaatccgttgattggctgagcactcgccgccctgcgggcgctcgcgacaagatcaattacattgcgcgccgcctgggcaaagtcggtacctttgagcttccaggcgaacaaagcttgtcgacgaaaaaagccggtctccaatcgtatgcagtgctcgttaacaaagagaaccgtggaaccagcatcaagctgtgggttgcgttcggcatcgtgatgttcggcttctacttcgccaacacttggaccccgaagctgctcgtggaaaccggaatgtcagaacagcagggcatcatcggtggtttgatgttgtccatgggtggagcattcggttccctgctctacggtttcctcaccaccaagttcagctcccgaaacacactgatgaccttcatggtgctgtccggcctgacgctgatcctgttcatttcctccacctctgttccatccatcgcgtttgccagcggcgttgtcgtgggcatgctgatcaatggttgtgtggctggtctgtacaccctgtccccacagctgtactccgctgaagtacgcaccactggtgtgggcgctgcgattggtatgggtcgtgtcggtgcgatttccgcgccactgctggtgggtagcctgctggattctggctggtccccaacgcagctgtatgttggtgtggcagtgattgttattgccggtgcaaccgcattgattgggatgcgcactcaggcagtagccgtcgaaaagcagcctgaagccctagcgaccaaatag

SEQ ID NO: 26 - protein, 475 aa, Corynebacterium glutamicum
MRLRVSSSLLPFLVPNLDHYGRPLLKEPGMDIRQTINDTAMSRYQWFIVFIAVLLNALDGFDVLAMSFTANAVTEEFGLSGSQLGVLLSSALFGMTAGSLLFGPIGDRFGRKNALMIALLFNVVGLVLSATAQSAGQLGVWRLITGIGIGGILACITVVISEFSNNKNRGMAMSIYAAGYGIGASLGGFGAAQLIPTFGWRSVFAAGAIATGIATIATFFFLPESVDWLSTRRPAGARDKINYIARRLGKVGTFELPGEQSLSTKKAGLQSYAVLVNKENRGTSIKLWVAFGIVMFGFYFANTWTPKLLVETGMSEQQGIIGGLMLSMGGAFGSLLYGFLTTKFSSRNTLMTFMVLSGLTLILFISSTSVPSIAFASGVVVGMLINGCVAGLYTLSPQLYSAEVRTTGVGAAIGMGRVGAISAPLLVGSLLDSGWSPTQLYVGVAVIVIAGATALIGMRTQAVAVEKQPEALATK

SEQ ID NO: 27 - DNA, 1296 bp, Corynebacterium glutamicum
gtgtcaacgaccaccccaacccgcgcaaccaaaagtgtcggaacagttctcgcactcctgtggttcgcaattgtcctcgacggctttgacctagtcgtcctgggcgcaacaatcccgtccatgctggaggatcccgcgtgggatctcactgctggacaggccacacagatttccaccatcggcctcgtcggcatgaccatcggcgcactgaccattggtttcttaactgaccgtctgggtcgacgccgcgtcatgctgttctctgtggcagtgttttctgtattcaccctcctgctggcattcaccaccaacgtccagctcttcagcctgtggcgtttcctcgcaggtgttggccttggtggagcactccccaccgcaattgccatggtgaccgagtttcgccccggcaccaaagcgggctctgcatcaactaccttgatgaccggataccacgtcggggcagtagcaaccgctttccttggtctcttccttatcgacggctttggttggcactccatgttcatcgcaggcgctgtgccaggactactcctgctgccactgctgtatttcttccttccagaatccccgcagtacctcaaaatctccggcaagttggatgaggcgcaggcagttgcagcatcttatggactttccctggatgatgatcttgatcgcgaacacgaagaagaacttggcgagtcctcctcactttcctccctgttcaagccctcgttccgccgcaacaccctggcgatttggggcacctcattcatgggactcctcctggtctacggcctgaacacatggctgccacaaatcatgcgccaagcagactacgacatgggtaactccctgggcttcctcatggttcttaacatcggcgcagtgatcggcctttatattgcagggcgaattgccgataagaactcccctcgcaaaacagcactcgtatggttcgtgttctctgcatttttcctcgcactacttgctgtccggatgccactgatcggtctgtatggcatcgtgctgctcaccggcatctttgtgttcagctcccaggtactcatctacgccttcgttggtgagaatcaccctgccaagatgcgtgcaactgccatgggattctccgcaggaattggtcgcctcggcgcgatctcgggtccgttgctgggcggcctgcttgtcagtgccaaccttgcttacccatggggcttcttcgccttcgctggcgttggactgctgggcgcgctgattttctccgcatcgaagactctgaggcatcgcgagaacgcttag

SEQ ID NO: 28 - protein, 431 aa, Corynebacterium glutamicum
MSTTTPTRATKSVGTVLALLWFAIVLDGFDLVVLGATIPSMLEDPAWDLTAGQATQISTIGLVGMTIGALTIGFLTDRLGRRRVMLFSVAVFSVFTLLLAFTTNVQLFSLWRFLAGVGLGGALPTAIAMVTEFRPGTKAGSASTTLMTGYHVGAVATAFLGLFLIDGFGWHSMFIAGAVPGLLLLPLLYFFLPESPQYLKISGKLDEAQAVAASYGLSLDDDLDREHEEELGESSSLSSLFKPSFRRNTLAIWGTSFMGLLLVYGLNTWLPQIMRQADYDMGNSLGFLMVLNIGAVIGLYIAGRIADKNSPRKTALVWFVFSAFFLALLAVRMPLIGLYGIVLLTGIFVFSSQVLIYAFVGENHPAKMRATAMGFSAGIGRLGAISGPLLGGLLVSANLAYPWGFFAFAGVGLLGALIFSASKTLRHRENA

SEQ ID NO: 29 - DNA, 1131 bp, Corynebacterium glutamicum
atgacactgtccgaacgcaagctcaccaccaccgccaagattcttccccacccactcaacgcctggtacgtcgccgcttgggattatgaagtcacatctaaaaagcccatggccaggacaatcgccaacaaaccactcgctttgtaccgcaccaaagatggccgagccgttgcccttgcagacgcctgctggcaccgcctcgcaccgctatccaagggaaaactcgtgggcacagacggaatccaatgcccttatcacggcttggagtacaactccgcgggccgctgcatgaaaatgcccgcgcaggaaaccctcaacccgtcagcagccgtcaactcctaccccgtggtggaagcccaccgctttgtgtgggtgtggctgggcgatcccacattggcagatcccacccaagtacccgatatgcaccagatgagccaccccgaatgggcaggcgatggacgcaccatctccgctgactgcaactaccaattagtgctggacaacttgatggacctcacccacgaagaattcgtgcactcctccagcatcggccaagacgaacttagtgaatcagagttcgtggtcacccacactgaagattccgtgacggtcacccgctggatgcatgacatagatgcaccaccgttttggcaaaagaacatgaatgataagttcccaggatttgaaggcaaggtggatcgttggcagatcatccactactactacccttccaccatctgcattgatgttggtgtagcaaaggctggaaccggcgcgcaggaaggcgaccgcagccagggcgttaatgggtatgtaatgaacaccattaccccagattcagatcgttcctctcattacttctgggcattcatgcgcaactaccgcctggaaagccaaaccatcaccacccagctgcgcgacggtgtatccggtgtattcaaagaagacgaagacatgctgaccgctcagcaagatgccatcgacgccaacaccgactatgagttttacagcctcaacattgatgccggtggcatgtgggtgcgccgaatcctcgaggaagcactctccaaggaaggccgactggatatccccaccacattcccccgcgcaacaccgaagccggaggcataa

SEQ ID NO: 30 - protein, 376 aa, Corynebacterium glutamicum
MTLSERKLTTTAKILPHPLNAWYVAAWDYEVTSKKPMARTIANKPLALYRTKDGRAVALADACWHRLAPLSKGKLVGTDGIQCPYHGLEYNSAGRCMKMPAQETLNPSAAVNSYPVVEAHRFVWVWLGDPTLADPTQVPDMHQMSHPEWAGDGRTISADCNYQLVLDNLMDLTHEEFVHSSSIGQDELSESEFVVTHTEDSVTVTRWMHDIDAPPFWQKNMNDKFPGFEGKVDRWQIIHYYYPSTICIDVGVAKAGTGAQEGDRSQGVNGYVMNTITPDSDRSSHYFWAFMRNYRLESQTITTQLRDGVSGVFKEDEDMLTAQQDAIDANTDYEFYSLNIDAGGMWVRRILEEALSKEGRLDIPTTFPRATPKPEA

SEQ ID NO: 31 - DNA, 978 bp, Corynebacterium glutamicum
atgaactcgcaatggcaagatgcacatgttgtttccagcgaaatcatcgctgcagacattcgacgaatagaactatccccgaaatttgcgattccagtaaaacccggcgaacatctcaagatcatggtgcccctaaaaactggacaggaaaagagatcgtactccatcgttgacgctcgtcacgacggttcgactctcgccctgagcgtactcaaaaccagaaactcccgtggaggatctgagttcatgcatacgcttcgagctggagacacagttactgtctccaggccgtctcaggattttcctctccgcgtgggtgcgcctgagtatgtacttgttgccggcggaattggaatcacagcgatccgttcaatggcatctttattaaagaaattgggagcaaactaccgcattcatttcgcagcacgcagccttgatgccatggcttacaaagatgagctcgtggcagaacacggcgacaagctgcacctgcatctagattctgaaggcaccaccatcgatgtcccagcattgatcgaaaccttaaacccccacactgagctttatatgtgcggccccatccgcttgatggatgccatccggcgcgcatggaacacccgcggacttgaccccaccaatctgcgtttcgaaacgtttggaaacagtggatggttctccccagaggttttccacatccaagtaccagagctggggcttcacgccacagtcaacaaggatgaaagcatgctggaggctttgcaaaaggctggggcgaatatgatgtttgattgtcgaaaaggcgaatgtggtttgtgccaggttcgcgttctagaagtcgatggccaggttgatcaccgcgatgtgttcttctctgatcgtcaaaaagaatccgacgcaaaggcatgcgcctgcgtgtctcgagtagtctcctccccttcctcgtccccaacctcgaccattacggtcgccctctcctaa

SEQ ID NO: 32 - protein, 325 aa, Corynebacterium glutamicum
MNSQWQDAHVVSSEIIAADIRRIELSPKFAIPVKPGEHLKIMVPLKTGQEKRSYSIVDARHDGSTLALSVLKTRNSRGGSEFMHTLRAGDTVTVSRPSQDFPLRVGAPEYVLVAGGIGITAIRSMASLLKKLGANYRIHFAARSLDAMAYKDELVAEHGDKLHLHLDSEGTTIDVPALIETLNPHTELYMCGPIRLMDAIRRAWNTRGLDPTNLRFETFGNSGWFSPEVFHIQVPELGLHATVNKDESMLEALQKAGANMMFDCRKGECGLCQVRVLEVDGQVDHRDVFFSDRQKESDAKACACVSRVVSSPSSSPTSTITVALS

SEQ ID NO: 33 - DNA, 615 bp, Corynebacterium glutamicum
atgattgatacagggaagaacggcgagttccgctacgagcagtcgaatatcatcgatcagaacgaagccgagttcggcatcactccttcacagaccgtgggcccttacgtccacatcggtttgacccttgaaggtgcggagcatctcgtggagccaggttcggaaggcgcggtgtcctttactgtttccgcaactgatggcaacggcgaccccatcgcggatgccatgtttgaactgtggcaggccgatccagagggcatccacaactctgatttggatccaaaccgcacagcaccagcaaccgcagatggcttccgcgggcttggtcgcgcgatggcaaacgcgcagggtgaggcaacgttcaccactttggttccgggagcattcgcagatgaggcaccacacttcaaggttggtgtgttcgcccgtggcatgctggagcgtctgtacactcgcgcatacctgccagacgccgatttgagcaccgacccagttttggctgtggtcccagctgatcgacgtgacctcctggtggctcaaaagaccgatgatggattccgcttcgacatcactgtccaggctgaagacaatgaaaccccattttttggactctaa

SEQ ID NO: 34 - protein, 204 aa, Corynebacterium glutamicum
MIDTGKNGEFRYEQSNIIDQNEAEFGITPSQTVGPYVHIGLTLEGAEHLVEPGSEGAVSFTVSATDGNGDPIADAMFELWQADPEGIHNSDLDPNRTAPATADGFRGLGRAMANAQGEATFTTLVPGAFADEAPHFKVGVFARGMLERLYTRAYLPDADLSTDPVLAVVPADRRDLLVAQKTDDGFRFDITVQAEDNETPFFGL

SEQ ID NO: 35 - DNA, 693 bp, Corynebacterium glutamicum
atggacatcccacacttcgccccgacgggaggcgaatactccccactgcacttcccggagtaccggaccaccatcaagcgcaacccaagcaacgatctcatcatggttcctagtcgcctcggcgagtccacgggacctgtcttcggcgaccgcgacttgggagacatcgacaacgacatgaccaaggtgaacggtggcgaggctatcggccagcgcatcttcgttcacggccgtgtcctcggtttcgatggcaagccagttccgcacaccttggtcgaggcgtggcaggcaaacgccgcaggccgttaccgccacaagaatgactcctggccagcgccactggatccacacttcaacggtgttgcacgtactctcaccgacaaggacggccagtaccacttctggaccgttatgccaggtaattacccttggggtaaccaccacaacgcatggcgcccggcgcacattcacttctcgctctatggtcgtcagtttacggagcgtctggtcacccagatgtacttcccgaacgatccattgttcttccaggatccgatctacaacgcggtgccaaagggtgcacgtgagcgcatgatcgcaacgttcgactatgacgagacccgtgaaaacttcgcgcttggttacaagttcgacatcgtccttcgtggccgcaacgccaccccatttgagtaa

SEQ ID NO: 36 - protein, 230 aa, Corynebacterium glutamicum
MDIPHFAPTGGEYSPLHFPEYRTTIKRNPSNDLIMVPSRLGESTGPVFGDRDLGDIDNDMTKVNGGEAIGQRIFVHGRVLGFDGKPVPHTLVEAWQANAAGRYRHKNDSWPAPLDPHFNGVARTLTDKDGQYHFWTVMPGNYPWGNHHNAWRPAHIHFSLYGRQFTERLVTQMYFPNDPLFFQDPIYNAVPKGARERMIATFDYDETRENFALGYKFDIVLRGRNATPFE

SEQ ID NO: 37 - DNA, 1164 bp, Escherichia coli
atgaacaactttaatctgcacaccccaacccgcattctgtttggtaaaggcgcaatcgctggtttacgcgaacaaattcctcacgatgctcgcgtattgattacctacggcggcggcagcgtgaaaaaaaccggcgttctcgatcaagttctggatgccctgaaaggcatggacgtgctggaatttggcggtattgagccaaacccggcttatgaaacgctgatgaacgccgtgaaactggttcgcgaacagaaagtgactttcctgctggcggttggcggcggttctgtactggacggcaccaaatttatcgccgcagcggctaactatccggaaaatatcgatccgtggcacattctgcaaacgggcggtaaagagattaaaagcgccatcccgatgggctgtgtgctgacgctgccagcaaccggttcagaatccaacgcaggcgcggtgatctcccgtaaaaccacaggcgacaagcaggcgttccattctgcccatgttcagccggtatttgccgtgctcgatccggtttatacctacaccctgccgccgcgtcaggtggctaacggcgtagtggacgcctttgtacacaccgtggaacagtatgttaccaaaccggttgatgccaaaattcaggaccgtttcgcagaaggcattttgctgacgctaatcgaagatggtccgaaagccctgaaagagccagaaaactacgatgtgcgcgccaacgtcatgtgggcggcgactcaggcgctgaacggtttgattggcgctggcgtaccgcaggactgggcaacgcatatgctgggccacgaactgactgcgatgcacggtctggatcacgcgcaaacactggctatcgtcctgcctgcactgtggaatgaaaaacgcgataccaagcgcgctaagctgctgcaatatgctgaacgcgtctggaacatcactgaaggttccgatgatgagcgtattgacgccgcgattgccgcaacccgcaatttctttgagcaattaggcgtgccgacccacctctccgactacggtctggacggcagctccatcccggctttgctgaaaaaactggaagagcacggcatgacccaactgggcgaaaatcatgacattacgttggatgtcagccgccgtatatacgaagccgcccgctaa

SEQ ID NO: 38 - protein, 387 aa, Escherichia coli
MNNFNLHTPTRILFGKGAIAGLREQIPHDARVLITYGGGSVKKTGVLDQVLDALKGMDVLEFGGIEPNPAYETLMNAVKLVREQKVTFLLAVGGGSVLDGTKFIAAAANYPENIDPWHILQTGGKEIKSAIPMGCVLTLPATGSESNAGAVISRKTTGDKQAFHSAHVQPVFAVLDPVYTYTLPPRQVANGVVDAFVHTVEQYVTKPVDAKIQDRFAEGILLTLIEDGPKALKEPENYDVRANVMWAATQALNGLIGAGVPQDWATHMLGHELTAMHGLDHAQTLAIVLPALWNEKRDTKRAKLLQYAERVWNITEGSDDERIDAAIAATRNFFEQLGVPTHLSDYGLDGSSIPALLKKLEEHGMTQLGENHDITLDVSRRIYEAAR

SEQ ID NO: 39 - DNA, 1062 bp, Corynebacterium glutamicum
atgagcatccaagtaaaagcactccagaaaaccggccccgaagcacctttcgaggtcaaaatcattgagcgtcgtgagcctcgcgctgacgacgtagttatcgacatcaaagctgccggcatctgccacagcgatatccacaccatccgcaacgaatggggcgaggcacacttcccgctcaccgtcggccacgaaatcgcaggcgttgtctctgcggttggctccgatgtaaccaagtggaaagtcggcgaccgcgttggcgtcggctgcctagttaactcctgcggcgaatgtgaacagtgtgtcgcgggatttgaaaacaactgccttcgcggaaacgtcggaacctacaactccgacgacgtcgacggcaccatcacgcaaggtggctacgccgaaaaggtagtggtcaacgaacgtttcctctgcagcatcccagaggaactcgacttcgatgtcgcagcaccactgctgtgcgcaggcatcaccacctactccccgatcgctcgctggaacgttaaagaaggcgacaaagtagcagtcatgggcctcggcgggctcggccacatgggtgtccaaatcgccgcagccaagggcgctgacgttaccgttctgtcccgttccctgcgcaaggctgaacttgccaaggaactcggcgcagctcgcacgcttgcgacttctgatgaggatttcttcaccgaacacgccggtgaattcgacttcatcctcaacaccattagcgcatccatcccagtcgacaagtacctgagccttctcaagccacacggtgtcatggctgttgtcggtctgccaccagagaagcagccactgagcttcggtgcgctcatcggcggcggaaaagtcctcaccggatccaacattggcggcatccctgaaacccaggaaatgctcgacttctgtgcaaaacacggcctcggcgcgatgatcgaaactgtcggcgtcaacgatgttgatgcagcctacgaccgcgttgttgccggcgacgttcagttccgcgttgtcattgatactgcttcgtttgcagaggtagaggcggtttag

SEQ ID NO: 40 - protein, 353 aa, Corynebacterium glutamicum
MSIQVKALQKTGPEAPFEVKIIERREPRADDVVIDIKAAGICHSDIHTIRNEWGEAHFPLTVGHEIAGVVSAVGSDVTKWKVGDRVGVGCLVNSCGECEQCVAGFENNCLRGNVGTYNSDDVDGTITQGGYAEKVVVNERFLCSIPEELDFDVAAPLLCAGITTYSPIARWNVKEGDKVAVMGLGGLGHMGVQIAAAKGADVTVLSRSLRKAELAKELGAARTLATSDEDFFTEHAGEFDFILNTISASIPVDKYLSLLKPHGVMAVVGLPPEKQPLSFGALIGGGKVLTGSNIGGIPETQEMLDFCAKHGLGAMIETVGVNDVDAAYDRVVAGDVQFRVVIDTASFAEVEAV

SEQ ID NO: 41 - DNA, 1113 bp, Corynebacterium glutamicum
gtgtccatgagcactgtcgtgcctggaattgtcgccctgtccaagggggcaccggtagaaaaagtaaacgttgttgtccctgatccaggtgctaacgatgtcatcgtcaagattcaggcctgcggtgtgtgccacaccgacttggcctaccgcgatggcgatatttcagatgagttcccttacctcctcggccacgaggcagcaggtattgttgaggaggtaggcgagtccgtcacccacgttgaggtcggcgatttcgtcatcttgaactggcgtgcagtgtgcggcgagtgccgtgcatgtaagaagggcgagccaaagtactgctttaacacccacaacgcatctaagaagatgaccctggaagacggcaccgagctgtccccagcactgggtattggcgcgttcttggaaaagaccctggtccacgaaggccagtgcaccaaggttaaccctgaggaagatccagcagcagctggccttctgggttgcggcatcatggcaggtcttggtgctgcggtaaacaccggtgatattaagcgcggcgagtccgtggcagtcttcggccttggtggcgtgggcatggcagctattgctggcgccaagattgctggtgcatcgaagattattgctgttgatatcgatgagaagaagttggagtgggcgaaggaattcggcgcaacccacaccattaattcctctggtcttggtggcgagggtgatgcctctgaggtcgtggcaaaggttcgtgagctcactgatggtttcggtactgacgtctccatcgatgcggtaggcatcatgccgacctggcagcaggcgttttactcccgtgatcatgcaggccgcatggtgatggtgggcgttccaaacctgacgtctcgcgtagatgttcctgcgattgatttttacggtcgcggtggctctgtgcgccctgcatggtacggcgactgcctgcctgagcgtgatttcccaacttatgtggatctgcacctgcagggtcgtttcccgctggataagtttgtttctgagcgtattggtcttgatgatgttgaagaggctttcaacaccatgaaggctggcgacgtgctgcgttctgtggtggagatctaa

SEQ ID NO: 42 - protein, 370 aa, Corynebacterium glutamicum
MSMSTVVPGIVALSKGAPVEKVNVVVPDPGANDVIVKIQACGVCHTDLAYRDGDISDEFPYLLGHEAAGIVEEVGESVTHVEVGDFVILNWRAVCGECRACKKGEPKYCFNTHNASKKMTLEDGTELSPALGIGAFLEKTLVHEGQCTKVNPEEDPAAAGLLGCGIMAGLGAAVNTGDIKRGESVAVFGLGGVGMAAIAGAKIAGASKIIAVDIDEKKLEWAKEFGATHTINSSGLGGEGDASEVVAKVRELTDGFGTDVSIDAVGIMPTWQQAFYSRDHAGRMVMVGVPNLTSRVDVPAIDFYGRGGSVRPAWYGDCLPERDFPTYVDLHLQGRFPLDKFVSERIGLDDVEEAFNTMKAGDVLRSVVEI

SEQ ID NO: 43 - DNA, 1047 bp, Corynebacterium glutamicum
gtgagttttatgaccactgctgcaccccaagaatttaccgctgctgttgttgaaaaattcggtcatgacgtgaccgtgaaggatattgaccttccaaagccagggccacaccaggcattggtgaaggtactcacctccggcatctgccacaccgacctccacgccttggagggcgattggccagtaaagccggaaccaccattcgtaccaggacacgaaggtgtaggtgaagttgttgagctcggaccaggtgaacacgatgtgaaggtcggcgatattgtcggcaatgcgtggctctggtcagcgtgcggcacctgcgaatactgcatcacaggcagggaaactcagtgtaacgaagctgagtacggtggctacacccaaaatggatccttcggccagtacatgctggtggatacccgatacgccgctcgcatcccagacggcgtggactacctcgaagcagcgccaattctgtgtgcaggcgtgactgtctacaaggcactcaaagtctctgaaacccgcccgggccaattcatggtgatctccggtgtcggcggacttggccacatcgcagtccaatacgcagcggcgatgggcatgcgtgtcattgcggtagatattgccgaggacaagctggaacttgcccgtaagcacggtgcggaatttaccgtgaatgcgcgtaatgaagatccaggcgaagctgtacagaagtacaccaacggtggcgcacacggcgtgcttgtgactgcagttcacgaggcagcattcggccaggcactggatatggctcgacgtgcaggaacaattgtgttcaacggtctgccaccgggagagttcccagcatccgtgttcaacatcgtattcaagggcctgaccatccgtggatccctcgtgggaacccgccaagacttggccgaagcgctcgatttctttgcacgcggactaatcaagccaaccgtgagtgagtgctccctcgatgaggtcaatggagttcttgaccgcatgcgaaacggcaagatcgatggtcgtgtggcgattcgtttctaa

SEQ ID NO: 44 - protein, 348 aa, Corynebacterium glutamicum
MSFMTTAAPQEFTAAVVEKFGHDVTVKDIDLPKPGPHQALVKVLTSGICHTDLHALEGDWPVKPEPPFVPGHEGVGEVVELGPGEHDVKVGDIVGNAWLWSACGTCEYCITGRETQCNEAEYGGYTQNGSFGQYMLVDTRYAARIPDGVDYLEAAPILCAGVTVYKALKVSETRPGQFMVISGVGGLGHIAVQYAAAMGMRVIAVDIAEDKLELARKHGAEFTVNARNEDPGEAVQKYTNGGAHGVLVTAVHEAAFGQALDMARRAGTIVFNGLPPGEFPASVFNIVFKGLTIRGSLVGTRQDLAEALDFFARGLIKPTVSECSLDEVNGVLDRMRNGKIDGRVAIRF

SEQ ID NO: 45 - DNA, 1020 bp, Corynebacterium glutamicum
atgcccaaatacattgccatgcaggtatccgaatccggtgcaccgttagccgcgaatctcgtgcaacctgctccgttgaaatcgagggaagtccgcgtggaaatcgctgctagtggtgtgtgccatgcagatattggcacggcagcagcatcggggaagcacactgtttttcctgttacccctggtcatgagattgcaggaaccatcgcggaaattggtgaaaacgtatctcggtggacggttggtgatcgcgttgcaatcggttggtttggtggcaattgcggtgactgcgctttttgtcgtgcaggtgatcctgtgcattgcagagagcggaagattcctggcgtttcttatgcgggtggttgggcacagaatattgttgttccagcggaggctcttgctgcgattccagatggcatggacttttacgaggccgccccgatgggctgcgcaggtgtgacaacattcaatgcgttgcgaaacctgaagctggatcccggtgcggctgtcgcggtctttggaatcggcggtttagtgcgcctagctattcagtttgctgcgaaaatgggttatcgaaccatcaccatcgcccgcggtttagagcgtgaggagctagctaggcaacttggcgccaaccactacatcgatagcaatgatctgcaccctggccaggcgttatttgaacttggcggggctgacttgatcttgtctactgcgtccaccacggagcctctttcggagttgtctaccggtctttctattggcgggcagctaaccattatcggagttgatgggggagatatcaccgtttcggcagcccaattgatgatgaaccgtcagatcatcacaggtcacctcactggaagtgcgaatgacacggaacagactatgaaatttgctcatctccatggcgtgaaaccgcttattgaacggatgcctctcgatcaagccaacgaggctattgcacgtatttcagctggtaaaccacgtttccgtattgtcttggagccgaattcataa

SEQ ID NO: 46 - protein, 339 aa, Corynebacterium glutamicum
MPKYIAMQVSESGAPLAANLVQPAPLKSREVRVEIAASGVCHADIGTAAASGKHTVFPVTPGHEIAGTIAEIGENVSRWTVGDRVAIGWFGGNCGDCAFCRAGDPVHCRERKIPGVSYAGGWAQNIVVPAEALAAIPDGMDFYEAAPMGCAGVTTFNALRNLKLDPGAAVAVFGIGGLVRLAIQFAAKMGYRTITIARGLEREELARQLGANHYIDSNDLHPGQALFELGGADLILSTASTTEPLSELSTGLSIGGQLTIIGVDGGDITVSAAQLMMNRQIITGHLTGSANDTEQTMKFAHLHGVKPLIERMPLDQANEAIARISAGKPRFRIVLEPNS

SEQ ID NO: 47 - DNA, 879 bp, Corynebacterium glutamicum
atgcaaacccttgctgctattgttcgtgccacgaagcaaccttttgagatcaccaccattgatctggatgcaccacgaccagatgaagttcaaatccgtgttattgctgccggagtgcgccacactgacgcaattgttcgtgatcagatttacccaacttttcttcccgcagttttcggccacgaaggcgccggagtagttgtcgccgtgggttctgcagtcacctcggtgaaaccagatgacaaggtagtgctgggattcaactcttgtggccagtgcttgaagtgtttgggcggtaagcctgcgtactgtgagaaattctatgaccgcaacttcgcatgcacccgcgatgccgggcacactactttgtttacccgtgcaacaaaagagcaggcagaggccatcatcgacacccttgatgatgttttctacgatgcggatgcgggtttcctggcatacccagcaactcccccagaggcttcgggagtaagcgtgttggttgtcgcggctggtacctctgatctcccccaagcaaaggaagcactacacactgcctcctacttggggcgctccacctcactgattgttgattttggagtggctggcatccaccgcctgctttcatacgaagaagaactccgcgctgcgggcgtgctcatcgttgccgctggaatggatggtgcgctacccggagttgtcgcaggcttagtgtccgcacctgtcgtcgcactgccaacctccgtgggatacggcgcaggtgctggaggaatcgcaccacttctgaccatgcttaacgcctgcgcgccgggagttggagtggtcaacattgataacggctatggagcaggacacctggctgcgcagattgcggcgaggtaa

SEQ ID NO: 48 - protein, 292 aa, Corynebacterium glutamicum
MQTLAAIVRATKQPFEITTIDLDAPRPDEVQIRVIAAGVRHTDAIVRDQIYPTFLPAVFGHEGAGVVVAVGSAVTSVKPDDKVVLGFNSCGQCLKCLGGKPAYCEKFYDRNFACTRDAGHTTLFTRATKEQAEAIIDTLDDVFYDADAGFLAYPATPPEASGVSVLVVAAGTSDLPQAKEALHTASYLGRSTSLIVDFGVAGIHRLLSYEEELRAAGVLIVAAGMDGALPGVVAGLVSAPVVALPTSVGYGAGAGGIAPLLTMLNACAPGVGVVNIDNGYGAGHLAAQIAAR

SEQ ID NO: 49 - DNA, 819 bp, Escherichia coli
atggaaacctatgctgtttttggtaatccgatagcccacagcaaatcgccattcattcatcagcaatttgctcagcaactgaatattgaacatccctatgggcgcgtgttggcacccatcaatgatttcatcaacacactgaacgctttctttagtgctggtggtaaaggtgcgaatgtgacggtgccttttaaagaagaggcttttgccagagcggatgagcttactgaacgggcagcgttggctggtgctgttaataccctcatgcggttagaagatggacgcctgctgggtgacaataccgatggtgtaggcttgttaagcgatctggaacgtctgtcttttatccgccctggtttacgtattctgcttatcggcgctggtggagcatctcgcggcgtactactgccactcctttccctggactgtgcggtgacaataactaatcggacggtatcccgcgcggaagagttggctaaattgtttgcgcacactggcagtattcaggcgttgagtatggacgaactggaaggtcatgagtttgatctcattattaatgcaacatccagtggcatcagtggtgatattccggcgatcccgtcatcgctcattcatccaggcatttattgctatgacatgttctatcagaaaggaaaaactccttttctggcatggtgtgagcagcgaggctcaaagcgtaatgctgatggtttaggaatgctggtggcacaggcggctcatgcctttcttctctggcacggtgttctgcctgacgtagaaccagttataaagcaattgcaggaggaattgtccgcgtga

SEQ ID NO: 50 - protein, 272 aa, Escherichia coli
METYAVFGNPIAHSKSPFIHQQFAQQLNIEHPYGRVLAPINDFINTLNAFFSAGGKGANVTVPFKEEAFARADELTERAALAGAVNTLMRLEDGRLLGDNTDGVGLLSDLERLSFIRPGLRILLIGAGGASRGVLLPLLSLDCAVTITNRTVSRAEELAKLFAHTGSIQALSMDELEGHEFDLIINATSSGISGDIPAIPSSLIHPGIYCYDMFYQKGKTPFLAWCEQRGSKRNADGLGMLVAQAAHAFLLWHGVLPDVEPVIKQLQEELSA

SEQ ID NO: 51 - DNA, 35 bp, Artificial Sequence
  primer
cggtacccggggatccttacttccgcgtatccaac

SEQ ID NO: 52 - DNA, 41 bp, Artificial Sequence
  primer
ctaggaatcgcggccggtgaactcctaaagaactatataac

SEQ ID NO: 53 - DNA, 20 bp, Artificial Sequence
  primer
ggccgcgattcctagcatgc

SEQ ID NO: 54 - DNA, 35 bp, Artificial Sequence
  primer
ccaagcttgcatgccagtcatcatcaacggtgccg

SEQ ID NO: 55 - DNA, 21 bp, Artificial Sequence
  primer
atctccgcagaagacgtactg

SEQ ID NO: 56 - DNA, 20 bp, Artificial Sequence
  primer
tccgatcatgtatgacctcc

SEQ ID NO: 57 - DNA, 36 bp, Artificial Sequence
  primer
cggtacccggggatcggcatagtgcttccaacgctc

SEQ ID NO: 58 - DNA, 36 bp, Artificial Sequence
  primer
tagctccactcaagattcctcgatattacctacagg

SEQ ID NO: 59 - DNA, 20 bp, Artificial Sequence
  primer
tcttgagtggagctagggcc

SEQ ID NO: 60 - DNA, 37 bp, Artificial Sequence
  primer
ccaagcttgcatgcccatatagagcccaggagctctc

SEQ ID NO: 61 - DNA, 23 bp, Artificial Sequence
  primer
cgccgcaaagtccaaatagaaag

SEQ ID NO: 62 - DNA, 20 bp, Artificial Sequence
  primer
ggattcttcctgaactcagc

SEQ ID NO: 63 - DNA, 36 bp, Artificial Sequence
  primer
cggtacccggggatcgggctcgtcctgaaattgcac

SEQ ID NO: 64 - DNA, 35 bp, Artificial Sequence
  primer
tccgtcgtgagccatgttgtgcccacgagactacc

SEQ ID NO: 65 - DNA, 20 bp, Artificial Sequence
  primer
atggctcacgacggattgcg

SEQ ID NO: 66 - DNA, 36 bp, Artificial Sequence
  primer
ccaagcttgcatgcccggttgcagccttcataaacg

SEQ ID NO: 67 - DNA, 21 bp, Artificial Sequence
  primer
agaccaatgagtacccaaccg

SEQ ID NO: 68 - DNA, 20 bp, Artificial Sequence
  primer
tcagcgtctggctcagctac

SEQ ID NO: 69 - DNA, 36 bp, Artificial Sequence
  primer
cggtacccggggatcaaccccagctcaaataacacc

SEQ ID NO: 70 - DNA, 37 bp, Artificial Sequence
  primer
tttcaacacaatccgtccttctcgcttggattacttg

SEQ ID NO: 71 - DNA, 23 bp, Artificial Sequence
  primer
cggattgtgttgaaattgctctg

SEQ ID NO: 72 - DNA, 35 bp, Artificial Sequence
  primer
ccaagcttgcatgcctcaccacgggaatcttcagg

SEQ ID NO: 73 - DNA, 20 bp, Artificial Sequence
  primer
ccggactggggtgtgttttg

SEQ ID NO: 74 - DNA, 20 bp, Artificial Sequence
  primer
cccggaaaatacggtatagc

SEQ ID NO: 75 - DNA, 35 bp, Artificial Sequence
  primer
ccaagcttgcatgccccatcgcattgccgaaaagc

SEQ ID NO: 76 - DNA, 35 bp, Artificial Sequence
  primer
aaagatcgggtcaatgcagttcgcggggcgaacat

SEQ ID NO: 77 - DNA, 35 bp, Artificial Sequence
  primer
cgccccgcgaactgcattgacccgatctttatacc

SEQ ID NO: 78 - DNA, 35 bp, Artificial Sequence
  primer
cggtacccggggatcaacgttgacggtgatgccat

SEQ ID NO: 79 - DNA, 25 bp, Artificial Sequence
  primer
gaaatgtcatacttcagccatcagg

SEQ ID NO: 80 - DNA, 25 bp, Artificial Sequence
  primer
tgcgagtgatgaaatcctgaaactt

SEQ ID NO: 81 - DNA, 35 bp, Artificial Sequence
  primer
ccaagcttgcatgcctttcgcggtgaatcaaccca

SEQ ID NO: 82 - DNA, 35 bp, Artificial Sequence
  primer
caggtcaaagctaaggcattgtctgtaaatgggca

SEQ ID NO: 83 - DNA, 35 bp, Artificial Sequence
  primer
ctaaggggtttagcaatgcccaatcaggcccactt

SEQ ID NO: 84 - DNA, 35 bp, Artificial Sequence
  primer
cggtacccggggatcttagggtacgagggtaagtg

SEQ ID NO: 85 - DNA, 93 bp, Artificial Sequence
  DNA fragment of P2 promoter
cttagctttgacctgcacaaatagttgcaaattgtcccacatacacataaagtagcttgcgtatttaaaattatgaacctaaggggtttagca

SEQ ID NO: 86 - DNA, 35 bp, Artificial Sequence
  primer
atttacagacaatgccttagctttgacctgcacaa

SEQ ID NO: 87 - DNA, 31 bp, Artificial Sequence
  primer
ggcctgattgggcattgctaaaccccttagg

SEQ ID NO: 88 - DNA, 1686 bp, Corynebacterium glutamicum
atgacaacaaccaccggaagtgcccggccagcacgtgccgccaggaagcctaagcccgaaggccaatggaaaatcgacggcaccgagccgcttaaccatgccgaggaaattaagcaagaagaacccgcttttgctgtcaagcagcgggtcattgatatttactccaagcagggtttttcttccattgcaccggatgacattgccccacgctttaagtggttgggcatttacacccagcgtaagcaggatctgggcggtgaactgaccggtcagcttcctgatgatgagctgcaggatgagtacttcatgatgcgtgtgcgttttgatggcggactggcttcccctgagcgcctgcgtgccgtgggtgaaatttctagggattatgctcgttccaccgcggacttcaccgaccgccagaacattcagctgcactggattcgtattgaagatgtgcctgcgatctgggagaagctagaaaccgtcggactgtccaccatgcttggttgcggtgacgttccacgtgttatcttgggctccccagtttctggcgtagctgctgaagagctgatcgatgccaccccggctatcgatgcgattcgtgagcgctacctagacaaggaagagttccacaaccttcctcgtaagtttaagactgctatcactggcaaccagcgccaggatgttacccacgaaatccaggacgtttccttcgttccttcgattcacccagaattcggcccaggatttgagtgctttgtgggcggcggcctgtccaccaacccaatgcttgctcagccacttggttcttggattccacttgatgaggttccagaagtgtgggctggcgtcgccggaattttccgcgactacggcttccgacgcctgcgtaaccgtgctcgcctcaagttcttggtggcacagtggggtattgagaagttccgtgaagttcttgagaccgaatacctcgagcgcaagctgattgatggcccagttgttaccaccaaccctggctaccgtgaccacattggcattcacccacaaaaggacggcaagttctacctcggtgtgaagccaaccgttggacacaccaccggtgagcagctcattgccattgctgatgttgcagaaaagcacggcatcaccaggattcgtaccacggcggaaaaggaactgctcttcctcgatattgagcgagagaaccttactaccgttgcacgtgacctggatgaaatcggactgtactcttcaccttccgagttccgccgcggcatcatttcctgcaccggcttggagttctgcaagcttgcgcacgcaaccaccaagtcacgagcaattgagcttgtggacgaactggaagagcgactcggcgatttggatgttcccatcaagattgccctgaacggttgccctaactcttgtgcacgcacccaggtttccgacatcggattcaagggacagaccgtcactgatgctgacggcaaccgcgttgaaggtttccaggttcacctgggcggttccatgaacttggatccaaacttcggacgcaagctcaagggccacaaggttattgccgatgaagtgggagagtacgtcactcgcgttgttacccacttcaaggaacagcgccacgaggacgagcacttccgcgattgggtccagcgggccgctgaggaagatttggtgtga

SEQ ID NO: 89 - protein, 561 aa, Corynebacterium glutamicum
MTTTTGSARPARAARKPKPEGQWKIDGTEPLNHAEEIKQEEPAFAVKQRVIDIYSKQGFSSIAPDDIAPRFKWLGIYTQRKQDLGGELTGQLPDDELQDEYFMMRVRFDGGLASPERLRAVGEISRDYARSTADFTDRQNIQLHWIRIEDVPAIWEKLETVGLSTMLGCGDVPRVILGSPVSGVAAEELIDATPAIDAIRERYLDKEEFHNLPRKFKTAITGNQRQDVTHEIQDVSFVPSIHPEFGPGFECFVGGGLSTNPMLAQPLGSWIPLDEVPEVWAGVAGIFRDYGFRRLRNRARLKFLVAQWGIEKFREVLETEYLERKLIDGPVVTTNPGYRDHIGIHPQKDGKFYLGVKPTVGHTTGEQLIAIADVAEKHGITRIRTTAEKELLFLDIERENLTTVARDLDEIGLYSSPSEFRRGIISCTGLEFCKLAHATTKSRAIELVDELEERLGDLDVPIKIALNGCPNSCARTQVSDIGFKGQTVTDADGNRVEGFQVHLGGSMNLDPNFGRKLKGHKVIADEVGEYVTRVVTHFKEQRHEDEHFRDWVQRAAEEDLV

SEQ ID NO: 90 - DNA, 249 bp, Corynebacterium glutamicum
gtgagtcttcggaggaaacccaatcccaaccgcaaccaccctctgtactgcccatactgcgcgggagaagttcttttccccgatgagcaaacagaattcgcgtggttgtgtgcggattgcaccagagtttttgaagtgaaatatcacggccaggacgatccagtgcacaggccagcaccagcaaagtccacatcgcaagcattaaaagaatctctcgaaagacacaaaagaggtgagtcgcaacaatga

SEQ ID NO: 91 - protein, 82 aa, Corynebacterium glutamicum
MSLRRKPNPNRNHPLYCPYCAGEVLFPDEQTEFAWLCADCTRVFEVKYHGQDDPVHRPAPAKSTSQALKESLERHKRGESQQ

SEQ ID NO: 92 - DNA, 786 bp, Corynebacterium glutamicum
atgagctttcaactagttaacgccctgaaaaatactggttcggtaaaagatcccgagatctcacccgaaggacctcgcacgaccacaccgttgtcaccagaggtagcaaaacacaacgaggaactcgtcgaaaagcatgctgctgcgttgtatgacgccagcgcgcaagagatcctggaatggacagccgagcacacgccgggcgctattgcagtgaccttgagcatggaaaacaccgtgctggcggagctggctgcgcggcacctgccggaagctgatttcctctttttggacaccggttaccacttcaaggaaactcttgaagttgcccgccaggtagatgagcgttattcccagaagcttgtcaccgcgctgccaatcctcaagcgcacggagcaggattccatttatggtctcaacctgtaccgcagcaacccagcggcgtgctgccgaatgcgcaaagttgaaccgctggcggcgtcgttaagcccatacgctggctggatcaccggcctgcgccgcgctgatggcccaacccgtgctcaagcccctgcgctgagcttggatgccaccggcaggctcaagatttctccaattatcacctggtcattggaggaaaccaacgagttcattgcggacaacaacctcatcgatcacccacttacccatcagggttatccatcaattggatgcgaaacctgcacccttcctgttgctgaaggacaagaccctagggccggccgttgggctggaaacgccaagacagaatgcggacttcactcatga

SEQ ID NO: 93 - protein, 261 aa, Corynebacterium glutamicum
MSFQLVNALKNTGSVKDPEISPEGPRTTTPLSPEVAKHNEELVEKHAAALYDASAQEILEWTAEHTPGAIAVTLSMENTVLAELAARHLPEADFLFLDTGYHFKETLEVARQVDERYSQKLVTALPILKRTEQDSIYGLNLYRSNPAACCRMRKVEPLAASLSPYAGWITGLRRADGPTRAQAPALSLDATGRLKISPIITWSLEETNEFIADNNLIDHPLTHQGYPSIGCETCTLPVAEGQDPRAGRWAGNAKTECGLHS

SEQ ID NO: 94 - DNA, 954 bp, Corynebacterium glutamicum
ttgggctggaaacgccaagacagaatgcggacttcactcatgaccacaaccgttgcatcagaactttccccacaccttaaagatcttgaaaatgaatccatccacatcctccgcgaggtagctggccagtttgataaggtcggcctgctgttttccggcggtaaggattccgtcgtggtgtacgagcttgcgcgccgcgctttcgctccagctaacgtgccttttgaattgctgcacgtggacaccggccacaacttcccagaggttttggaattccgcgacaacctggtggagcgcaccggcgcccgcctgcgcgtagctaaagtccaggactggatcgatcgcggtgacctgcaggaacgcccagacggcacccgcaacccactgcagactgtccctttggtggagaccatcgctgagcagggctacgacgccgtgcttggtggcgctcgccgcgatgaggagcgtgcccgcgccaaggagcgtgtgttctctgtgcgtgactccttcggtggttgggatccacgccgtcagcgcccagagctgtggaccctctacaacggtggccacctgccaggcgaaaacatccgtgttttcccaatctccaactggactgaagctgacatctgggagtacatcggcgcccgtggcatcgaacttccaccgatctacttctcccacgaccgcgaagttttcgagcgcgacggcatgtggctgaccgcaggcgagtggggtggaccaaagaagggcgaggagatcgtcaccaagactgtccgctaccgcaccgtcggcgatatgtcctgcaccggtgctgtgctctcagaagcccgcaccattgacgatgtgatcgaagagatcgccacctccacccttaccgaacgtggcgcaacccgcgccgatgaccgcctcagcgaatccgcaatggaagaccgcaagaaggaaggctacttctga

SEQ ID NO: 95 - protein, 317 aa, Corynebacterium glutamicum
MGWKRQDRMRTSLMTTTVASELSPHLKDLENESIHILREVAGQFDKVGLLFSGGKDSVVVYELARRAFAPANVPFELLHVDTGHNFPEVLEFRDNLVERTGARLRVAKVQDWIDRGDLQERPDGTRNPLQTVPLVETIAEQGYDAVLGGARRDEERARAKERVFSVRDSFGGWDPRRQRPELWTLYNGGHLPGENIRVFPISNWTEADIWEYIGARGIELPPIYFSHDREVFERDGMWLTAGEWGGPKKGEEIVTKTVRYRTVGDMSCTGAVLSEARTIDDVIEEIATSTLTERGATRADDRLSESAMEDRKKEGYF

SEQ ID NO: 96 - DNA, 1302 bp, Corynebacterium glutamicum
atgactgctccaaccttgaataaagcatccgaaaagattgcatcacgcgagacccttcgtctgtgcaccgcaggttccgtagatgatggcaagtccaccttcgtcggccgcctcctgcacgacaccaagtctgttcttgctgatcagctagcttccgtagagcgcacctccgccgaccgcggcttcgaaggcctcgacctgtccctcctcgtcgacggcctgcgcgccgagcgtgagcagggcatcaccatcgacgttgcctaccgctacttcgccactgacaagcgcaccttcatcctggctgacaccccaggccacgtgcagtacacccgcaacaccgtcaccggcgtctccacctcccaggttgtagttttgcttgtcgacgcccgccacggcgtcgtcgagcagacccgccgccacctgtccgtatcggccctgctgggcgtgcgcacggtgatcctcgcagtcaacaaaattgaccttgttgattacagcgaagaagtcttccgcaacattgaaaaagaattcgtttctttggcttccgctttagatgtcaccgacacccacgtcgttccgatctccgcactcaagggcgacaacgttgcagaaccttccacccacatggactggtacgcgggaccaaccgtgctggaaatcctggaaaacgttgaagtttcccgcggccgtgcacacgacctgggcttccgcttcccaatccagtacgtcatccgcgagcacgcaaccgattaccgcggctacgccggcaccatcaacgctggttccatctccgtgggcgataccgtgcacctacctgaaggccgcaccacccaggtcacccacatcgattccgctgacggatccctccaaaccgcatcagttggagaagccgttgtcctgcgcctagcccaggaaatcgacctcatccgcggcgaactcatcgcaggctccgatcgcccagaatccgttcgttccttcaacgccactgtcgttggtctagcagatcgcactatcaaaccaggtgcagcagtcaaggtccgctacggcaccgagctggtccgcggacgcgtcgcagccatcgaacgagtcctcgacatcgacggcgtcaacgacaacgaagcaccagaaacctacggcctcaacgacatcgcgcacgtgcgcatcgatgttgcaggtgaattggaagttgaagattacgctgctcgtggcgcaattggctccttccttcttatcgatcaatcctccggcgacaccctcgctgccggtttggttggccaccgcctacgcaataactggtcgatctag

SEQ ID NO: 97 - protein, 433 aa, Corynebacterium glutamicum
MTAPTLNKASEKIASRETLRLCTAGSVDDGKSTFVGRLLHDTKSVLADQLASVERTSADRGFEGLDLSLLVDGLRAEREQGITIDVAYRYFATDKRTFILADTPGHVQYTRNTVTGVSTSQVVVLLVDARHGVVEQTRRHLSVSALLGVRTVILAVNKIDLVDYSEEVFRNIEKEFVSLASALDVTDTHVVPISALKGDNVAEPSTHMDWYAGPTVLEILENVEVSRGRAHDLGFRFPIQYVIREHATDYRGYAGTINAGSISVGDTVHLPEGRTTQVTHIDSADGSLQTASVGEAVVLRLAQEIDLIRGELIAGSDRPESVRSFNATVVGLADRTIKPGAAVKVRYGTELVRGRVAAIERVLDIDGVNDNEAPETYGLNDIAHVRIDVAGELEVEDYAARGAIGSFLLIDQSSGDTLAAGLVGHRLRNNWSI

SEQ ID NO: 98 - DNA, 900 bp, Corynebacterium glutamicum
ttggctccttccttcttatcgatcaatcctccggcgacaccctcgctgccggtttggttggccaccgcctacgcaataactggtcgatctagaccagttgctgtgaaggcaaggtgccggcttagatgccggcgcctagcctacatccagctaagaccccctttaggacacctcatgattcccctgattacgctttcccacggttcccgcaaaaagtccgcagctgcaggtattactgcgctgactcatgaggccggacgaatgctggaaacaccagccgtggaagcgcatttagagcttgctgaaccttcccttgatcaggttgtggcaacgctcagtgcggaaggcgtaaccagggcagcgttggttcctttgctgtttagcaatgcgtatcacgcaaagattgacgttcctgaggcagtaaaagatgcttcagaaaagtatggtgtggaacttctcgtgggtccgcatttgggcactggctccgatgtagccagcgtgcttgcgcagcggttgcgtgcggacgcccccacagatgcccatgtgattttgtattccgttggcagctcacacgtgtccgccaatgaatcagtcatcgatcttgcccacaccattgctctcctcactggcttttcggttgaggtggtgcccgctaccggtgggccaggtgccggcggcgccggagtaatagaggtggcctcgaaacacaaggccgtccacatcctgccgctgtttgttacggaaggtttgctgctggatcgggttattgatcaatccgccaacatcgcagctgccaccggcacgaactttacctattccgaacccctaactactgacctcgcaccacttgttgcagcccgttaccacgctgcattgagcgcactgctggcacatatctaa

SEQ ID NO: 99 - protein, 299 aa, Corynebacterium glutamicum
MAPSFLSINPPATPSLPVWLATAYAITGRSRPVAVKARCRLRCRRLAYIQLRPPLGHLMIPLITLSHGSRKKSAAAGITALTHEAGRMLETPAVEAHLELAEPSLDQVVATLSAEGVTRAALVPLLFSNAYHAKIDVPEAVKDASEKYGVELLVGPHLGTGSDVASVLAQRLRADAPTDAHVILYSVGSSHVSANESVIDLAHTIALLTGFSVEVVPATGGPGAGGAGVIEVASKHKAVHILPLFVTEGLLLDRVIDQSANIAAATGTNFTYSEPLTTDLAPLVAARYHAALSALLAHI

SEQ ID NO: 100 - DNA, 930 bp, Corynebacterium glutamicum
atgcagacattaatctttatcgccattgcaggcgtcgcagcacagcttgttgatggcggcctcggcatggggttcggcgtcacctcaaccaccatcctcatcatgctcgcaggtttaggccctgcgcaggcatccgccgtcgtgcacaccgcagaggttggaaccaccttagtttctggtttaagccactggaaatttggcaacgtggattggaaagtagttgtccggctcggtatccccggcgctatcggcgcatttgctggcgctaccttcttgtccaatatttccaccgaagcagcagcaccgatcacctccctgattcttgccctgatcggcatgaacctagtctggcgattcagcaagggacgcatccgccgcgactattccgatcgcccgcacagcaagggattcctcggcggactcggtattgtcggtggcttcgttgacgcgtccggtggcggcggatggggtccagtgaccacctctacgctgctgtctttgggacgcaccgaaccccgcaaagtagtcggcaccgtcaacaccgcagaattcttagtctccctagccgcaacattgggcttcgtcgtgggactgtgggatgacctagtagctaacctctctgcagttctcgcgttgctcatcggcggcgcaatcgcagcaccaatcggcgcctggatgatctctcgcgttaatgcaaccgtcctcggcggcttcgtgggcaccctgattgtcacactgaacctgccaaaggtgctcaatgtggttggccttgatttcatccccaccggcctcgtccaggtcaccgtcctcctcatcggcctgccgctgacgtacctcggcttccgccgctaccgcaaaaacctcctcaacgaaaccatctccagcgaggttgtctccgaaccacagggacaaaagattaaaagctcttaa

SEQ ID NO: 101 - protein, 309 aa, Corynebacterium glutamicum
MQTLIFIAIAGVAAQLVDGGLGMGFGVTSTTILIMLAGLGPAQASAVVHTAEVGTTLVSGLSHWKFGNVDWKVVVRLGIPGAIGAFAGATFLSNISTEAAAPITSLILALIGMNLVWRFSKGRIRRDYSDRPHSKGFLGGLGIVGGFVDASGGGGWGPVTTSTLLSLGRTEPRKVVGTVNTAEFLVSLAATLGFVVGLWDDLVANLSAVLALLIGGAIAAPIGAWMISRVNATVLGGFVGTLIVTLNLPKVLNVVGLDFIPTGLVQVTVLLIGLPLTYLGFRRYRKNLLNETISSEVVSEPQGQKIKSS

SEQ ID NO: 102 - DNA, 1374 bp, Corynebacterium glutamicum
atgacaactcccctgcgcgtagccatcatcggagctggccctgctggcatttacgcatccgacctcctcatccgcaatgaagagcgcgaagtgttcgttgaccttttcgagcaaatgcctgcaccgttcggactcatccgttacggcgttgcaccagaccacccacgcatcaagggcatcgttaagtccctgcacaacgtgttggacaagccacgcctgcgcctgctcggcaacattgaaatcggcaaagacatcaccgtcgaagaactccgcgactactacgacgcagttgtcttctccaccggtgcagttgcagaccgcgacctcaacatccccggaattgaagcagaaggttccttcggtgccggcgagttcgttggcttctacgacggcaacccacgcttcgagcgctcctgggatctgtctgcacagtccgtcgctgttatcggcgttggtaacgtcggcctcgatgtagcccgcatcctggctaagacaggcgacgagctcaaagtcaccgaaatttccgacaacgtctacgactccctcaaagaaaacaaggccactgaagtacacgttttcggacgtcgtggcccagcacaggtcaagttcaccccacaggaactcaaagaactcgaccactcccccaccatcaacgtggttgttgacccagaagacatcgactacgacggcgcctccgaagaagcccgccgcgcatccaaatcccaggacctggtctgccagatcctggaacagtacgcaatccgcgagccaaaggacgctccgcacaccctgcagatccacctctttgaaaacccagttgaggttcttcaaaaggacggcaaggttgttggcctgcgcaccgaacgcaccgcgctcgacggcaacggtggcgtaaacggcaccggcgaattcaaggactggccagttcaggctgtctaccgcgcagtcggctacaagtccgaccccatcgacggcgtcccattcgatgggaacaagcacgtcatccctaatgacggcggacatgtcctcaccgctccaggtgcagagccagtaccaggcctctacgccaccggctggatcaagcgtggaccaatcggtctgatcggcaacaccaagtctgatgccaaggaaaccaccgacatcctcatcaaggatgccgtcaccggtgtacttgaagccccaaagcaccagggcgaagaagccatcatcgagcttctcgattcccgcaacatcccattcaccacctgggaaggctggtacaaactcgacgcagcagagcgcgcactcggtgaagccgaaggccgcgagcgcaagaagattgttgattgggaagaaatggtccgccaggcccgcgaagctccagcaattgtctaa

SEQ ID NO: 103 - protein, 457 aa, Corynebacterium glutamicum
MTTPLRVAIIGAGPAGIYASDLLIRNEEREVFVDLFEQMPAPFGLIRYGVAPDHPRIKGIVKSLHNVLDKPRLRLLGNIEIGKDITVEELRDYYDAVVFSTGAVADRDLNIPGIEAEGSFGAGEFVGFYDGNPRFERSWDLSAQSVAVIGVGNVGLDVARILAKTGDELKVTEISDNVYDSLKENKATEVHVFGRRGPAQVKFTPQELKELDHSPTINVVVDPEDIDYDGASEEARRASKSQDLVCQILEQYAIREPKDAPHTLQIHLFENPVEVLQKDGKVVGLRTERTALDGNGGVNGTGEFKDWPVQAVYRAVGYKSDPIDGVPFDGNKHVIPNDGGHVLTAPGAEPVPGLYATGWIKRGPIGLIGNTKSDAKETTDILIKDAVTGVLEAPKHQGEEAIIELLDSRNIPFTTWEGWYKLDAAERALGEAEGRERKKIVDWEEMVRQAREAPAIV

SEQ ID NO: 104 - DNA, 1173 bp, Corynebacterium glutamicum
ttgtctatgattggctatggtttacctatgcccaatcaggcccacttctctgcgtcctttgcccgcccctctaccccggctgcaaagtgcatgcaccatatccgcctcggccagcaactcattagaaatgagctggtcgaggccacaggtctgtcccaaccgactgtcacccgcgcagtcaccgctttaatgcaggcaggtttggttcgtgaacgccctgatctcacactctcatcgggccctggtcgtcccaatattcctctagaactcgctccaagtccatggattcatgcaggcgtggcaatcggcaccaagtcttcctacgtcgctttgtttgataccaagggtcgcacccttcgtgatgccatactggaaatctcagcagctgatttagatccagacaccttcatcgaacacctcatcgctggtgtcaaccgcctcaccactggtcttgatctaccactggtaggtattggtgtggctacctcaggaaaagtcaccaacgcgggcgttgtcaccgcaagcaacttgggctgggatggcgttgatatcgccggccgtctgaactaccaattcagcgttccagcaaccgtggcatcagcaattcctgccatcgcagcttctgaactgcaggcttccccacttccccaccctgagcagccaactcccatcaccttgaccttctacgccgatgactctgtgggcgcggcctacagcaatgatttgggagtacatgtcattggaccactggctacaactcgtggatcaggtttggatactttgggcatggctgctgaagatgcgctgagcacccaaggtttcttaagcagggtttctgatcagggtatctttgccaacagccttggtgagctagtcaccattgctaaagacaatgaaaccgcacgggaattcctcaacgatcgcgcgaccctgctggctcacactgccgcagaagctgctgaaacagttaagccatccaccctggttctctcgggatcggcgttttccgaagatccacaaggtcggttggtgttcgcttcccaattgaagaaggaatacgacgcagacattgagctccgcttgatccccacccaccgggaaaatgtccgcgcagcagctcgcgcagtcgcacttgatcgactactcaacgagccacttaccctcgtaccctaa

SEQ ID NO: 105 - protein, 390 aa, Corynebacterium glutamicum
LSMIGYGLPMPNQAHFSASFARPSTPAAKCMHHIRLGQQLIRNELVEATGLSQPTVTRAVTALMQAGLVRERPDLTLSSGPGRPNIPLELAPSPWIHAGVAIGTKSSYVALFDTKGRTLRDAILEISAADLDPDTFIEHLIAGVNRLTTGLDLPLVGIGVATSGKVTNAGVVTASNLGWDGVDIAGRLNYQFSVPATVASAIPAIAASELQASPLPHPEQPTPITLTFYADDSVGAAYSNDLGVHVIGPLATTRGSGLDTLGMAAEDALSTQGFLSRVSDQGIFANSLGELVTIAKDNETAREFLNDRATLLAHTAAEAAETVKPSTLVLSGSAFSEDPQGRLVFASQLKKEYDADIELRLIPTHRENVRAAARAVALDRLLNEPLTLVP

SEQ ID NO: 106 - DNA, 1074 bp, Corynebacterium glutamicum
gtgttcatgcttgcacagcgaacactccccattcacatcaccgccccccacctgcccgtcgcgcgcgtatttcaccaaattcgcgccacagacgccgatcgcacctcgctgcaacgcgatcttgaactctcccaagctggcatcactcggcatgtatcagcgcttattgatgcaggtctcgtggaggaaacccgagtggattccggggcgcgctcggggcgaccgcgcacaaaattaggcatcgacggccgccatctcaccgcctggggagtgcacattggcctgcgcagcacggattttgcggtgtgcgatttagccggccgagtgattaggtatgagcgcgtggaccatgaagtttcacactccacgccgtcggaaacgctgaattttgtcgcacataggttacaaacattgagcgccggcttgcccgagccccgcaatgtgggcgtggcattatctgcccacttaagcgccaacggcaccgtcacttccgaagattatggctggtcagaggtggaaattgggatacacctccccttccccgccaccatcggatcaggtgttgcggcgatggccggttcggaaattatcaacgcgccactgacccaatccacgcagtccacgctgtatttctacgcccgcgaaatggtctcccacgcctggattttcaacggcgctgtccaccgccccaacagcggccgcacgccgacggcgttcggaaatacaaataccttaaaagatgcttttcgacgtggactcacaccaacaactttctccgatttagtccaactctcccacaccaacccgcttgcccgacagatcctcaacgagcgcgcccacaaacttgccgacgccgtaaccaccgccgttgatgttgtcgaccccgaagccgtcgtcttcgccggcgaagccttcaccctggatccggaaactcttcgcattgtggtgacccagctccgagcaaacaccggcagccaactgagaatccaacgcgcagacgcccacattctccgcaccgcggccatccaggtggcgctgcatccgatccgtcaagatccgttagcatttgtgtaa

SEQ ID NO: 107 - protein, 357 aa, Corynebacterium glutamicum
MFMLAQRTLPIHITAPHLPVARVFHQIRATDADRTSLQRDLELSQAGITRHVSALIDAGLVEETRVDSGARSGRPRTKLGIDGRHLTAWGVHIGLRSTDFAVCDLAGRVIRYERVDHEVSHSTPSETLNFVAHRLQTLSAGLPEPRNVGVALSAHLSANGTVTSEDYGWSEVEIGIHLPFPATIGSGVAAMAGSEIINAPLTQSTQSTLYFYAREMVSHAWIFNGAVHRPNSGRTPTAFGNTNTLKDAFRRGLTPTTFSDLVQLSHTNPLARQILNERAHKLADAVTTAVDVVDPEAVVFAGEAFTLDPETLRIVVTQLRANTGSQLRIQRADAHILRTAAIQVALHPIRQDPLAFV

SEQ ID NO: 108 - DNA, 2180 bp, Artificial Sequence
  promoter P2
tttcgcggtgaatcaacccacccgaacggcgatccttcgaagtattttgccgattgatcaattagcgtcggcaacatcactgaatatgctgctcatgcagaccggcgcaatcgttggcccgctgatcgcaggtgcgttgattccgctgatcggtttcgggtggctgtatttccttgatgttgtctccatcatccccacactgtgggctgtatggtcactgccttcaatcaagccatccggcaaggtcatgaaggccggtttcgccagtgtggtggatggcctgaagtatttggctggccaacccgtgttgttgatggtgatggtgctggatcttatcgccatgattttcggcatgccacgtgcgctttaccccgagatcgcggaagtgaacttcggtggtggtgacgccggtgcaacgatgctggcgttcatgtactcatccatggctgttggcgcagttcttggcggcgtgctgtctggttgggtttcccggattagccgccagggtgttgcagtttattggtgcatcatcgcctggggcgcagccgttgctttgggtggcgtagcaattgttgtcagccccggcgctgtgaccgcgtgggcgtggatgttcatcatcatgatggtcattggtggcatggctgacatgtttagctcggctgttcgaaatgctattttgcagcagtctgcagcggaacatgtgcagggccgaatccaaggtgtgtggatcatcgtcgtggtgggtggacctcgtttagctgacgtccttcacggttgggccgctgagcccttgggtgcaggttggacggtattatggggcggagtagcggtggttgtactcactgcaatttgtatggtggcggtgcctaaattctggaaatacgagaaaccaaaaattaccggcatctaaatacttatccatgcccatttacagacaatgccttagctttgacctgcacaaatagttgcaaattgtcccacatacacataaagtagcttgcgtatttaaaattatgaacctaaggggtttagcaatgcccaatcaggcccacttctctgcgtcctttgcccgcccctctaccccggctgcaaagtgcatgcaccatatccgcctcggccagcaactcattagaaatgagctggtcgaggccacaggtctgtcccaaccgactgtcacccgcgcagtcaccgctttaatgcaggcaggtttggttcgtgaacgccctgatctcacactctcatcgggccctggtcgtcccaatattcctctagaactcgctccaagtccatggattcatgcaggcgtggcaatcggcaccaagtcttcctacgtcgctttgtttgataccaagggtcgcacccttcgtgatgccatactggaaatctcagcagctgatttagatccagacaccttcatcgaacacctcatcgctggtgtcaaccgcctcaccactggtcttgatctaccactggtaggtattggtgtggctacctcaggaaaagtcaccaacgcgggcgttgtcaccgcaagcaacttgggctgggatggcgttgatatcgccggccgtctgaactaccaattcagcgttccagcaaccgtggcatcagcaattcctgccatcgcagcttctgaactgcaggcttccccacttccccaccctgagcagccaactcccatcaccttgaccttctacgccgatgactctgtgggcgcggcctacagcaatgatttgggagtacatgtcattggaccactggctacaactcgtggatcaggtttggatactttgggcatggctgctgaagatgcgctgagcacccaaggtttcttaagcagggtttctgatcagggtatctttgccaacagccttggtgagctagtcaccattgctaaagacaatgaaaccgcacgggaattcctcaacgatcgcgcgaccctgctggctcacactgccgcagaagctgctgaaacagttaagccatccaccctggttctctcgggatcggcgttttccgaagatccacaaggtcggttggtgttcgcttcccaattgaagaaggaatacgacgcagacattgagctccgcttgatccccacccaccgggaaaatgtccgcgcagcagctcgcgcagtcgcacttgatcgactactcaacgagccacttaccctcgtaccctaa

SEQ ID NO: 109 - DNA, 2247 bp, Artificial Sequence
  promoter P4
ccctcatgagttcaggggttagaaaagcaatgggatttggatgcggttcggttttggccgtcatcatggttatctcatttgttggatgggcgcttagcttcatggatggaacggcacctattcgccaactccagcaaatccctgaagatgttccgccggcgcgtggtgtagaagttccgcaaattgatacaggggcagatggacgcacgtcagatcatttgcgtttttgggcggaaccaattgctcaagatgctggtgtgtccgctcaagcgattgcggcttatggaaacgcagagctcattgcgagtactgcgtggcctggctgcaatctggggtggaataccttggcaggtatcggccaggtggaaacccgtcacggtacctacaacggcaaaatgttcgggggcagttccctggatgaaaatggagttgcaacccctccaatcatcggcgttccacttgatggttcaccggggtttgcggaaattcccgacactgatggtggggaattagatggcgatactgaatatgatcgcgcggtaggtcccatgcagttcattccggaaacgtggcgacttatgggattggatgcaaacggtgatggggtagcggaccccaaccaaattgatgacgcagcattgagtgccgcaaacctgttgtgttccaacgatcgtgacttgtccactcctgaaggatggaccgcagctgttcattcttacaacatgtctaatcagtatttgatggacgttcgagatgctgccgcgtcctacgctttacgacagccggcgatctaaaacttaacaagcgcaacccccgaaaatgtgagattatgtccggtcggacacgtgcgggctggggatatgggtagtttaataaatttataccacacagtctattgcaatagaccaagctgttcagtagggtgcatgggagaagaatttcctaataaaaactcttaaggacctccaagtggctgaaatcatgcacgtattcgctcgcgaaattctcgactcccgcggtaacccaaccgtcgaggcagaggttttccttgatgacggttcccacggtgtcgcaggtgttccatccggcgcatccaccggcgtccacgaggctcatgagctgcgtgacggtggcgatcgctacctgggcaagggcgttttgaaggcagttgaaaacgtcaacgaagaaatcggcgacgagctcgctggcctagaggctgacgatcagcgcctcatcgacgaagcaatgatcaagcttgatggcaccgccaacaagtcccgcctgggtgcaaacgcaatccttggtgtttccatggctgttgcaaaggctgctgctgattccgcaggcctcccactgttccgctacatcggtggaccaaacgcacacgttcttccagttccaatgatgaacatcatcaacggtggcgctcacgctgactccggtgttgacgttcaggaattcatgatcgctccaatcggtgcagagaccttctctgaggctctccgcaacggcgcagaggtctaccacgcactgaagtccgtcatcaaggaaaagggcctgtccaccggacttggcgatgagggcggcttcgctccttccgtcggctccacccgtgaggctcttgaccttatcgttgaggcaatcgagaaggctggcttcaccccaggcaaggacatcgctcttgctctggacgttgcttcctctgagttcttcaaggacggcacctaccacttcgaaggtggccagcactccgcagctgagatggcaaacgtttacgctgagctcgttgacgcgtacccaatcgtctccatcgaggacccactgcaggaagatgactgggagggttacaccaacctcaccgcaaccatcggcgacaaggttcagatcgttggcgacgacttcttcgtcaccaaccctgagcgcctgaaggagggcatcgctaagaaggctgccaactccatcctggttaaggtgaaccagatcggtaccctcaccgagaccttcgacgctgtcgacatggctcaccgcgcaggctacacctccatgatgtcccaccgttccggtgagaccgaggacaccaccattgctgacctcgcagttgcactcaactgtggccagatcaagactggtgctccagcacgttccgaccgtgtcgcaaagtacaaccagcttctccgcatcgagcagttgcttggcgacgccggcgtctacgcaggtcgcagcgcattcccacgctttcagggctaa

SEQ ID NO: 110 - DNA, 2192 bp, Artificial Sequence
  promoter P8
tcaccgagtctttgatcaagggtggcgcttttgactcccttggacacgcacgaaaaggcctcatgctggtcttcgaagatgccgttgattccgtcatcgctaccaaaaaagctgctgacaagggacaatttgatctctttgcagctttcgactcggataacaacgacgatgtggcaagtttcttccagatcaccgttcctgatgacgaatgggaccgtaagcatgagctcgcactcgagcgagaaatgctgggtctgtatgtttctggacacccactcgatggctatgaagatgccattgctgcccaggttgatacagcactgaccaccattgttgccggtgaactcaagcacggcgcagaagtgaccgtgggtggcattatctctggtgtggatcgacggttctccaagaaggacggttccccttgggcgattgtcaccattgaagatcacaacggcgcgtccgttgaattgttggtcttcaacaaggtgtattccatcgttggatccatgattgtggaagacaacatcattttggccaaggcacacatctccattcgagatgatcgtatgagccttttctgtgatgatctccgcgttccagagcttgggccaggaaacgggcaaggacttccgcttcgtttgtccatgcgtactgatcagtgcaccatgtccaacattgccaagctcaagcaggtgctggtggacaacaagggtgaatctgatgtgtacctcaatttgatcgatggggataactccacggtcatgattttgggtgatcacttaagagtcaaccgatccgcaagtttgatgggcgacctcaaggcaacgatggggccaggcatcctcggttaatcacatcacactgggattaccccgtgtaggggtgaaaacccgaatgtggctaaaacttttggaaacttaagttacctttaatcggaaacttattgaattcgggtgaggcaactgcaactctggacttaaagcatgagccagaaccgcatcaggaccactcacgttggttccttgccccgtaccccagagctacttgatgcaaacatcaagcgctctaacggtgagattggggaggaggaattcttccagatcctgcagtcttctgtagatgacgtgatcaagcgccaggttgacctgggtatcgacatcctcaacgagggcgaatacggccacgtcacctccggtgcagttgacttcggtgcatggtggaactactccttcacccgcctgggcggactgaccatgaccgataccgaccgttgggcaagccaggaagcagtgcgttccacccctggcaacatcaagctgaccagcttctctgatcgtcgcgaccgcgcattgttcagcgaagcatacgaggatccagtatctggcatcttcaccggccgcgcttctgtgggcaacccagagttcaccggacctattacctacattggccaggaagaaactcagacggatgttgatctgctgaagaagggcatgaacgcagcgggagctaccgacggcttcgttgcagcactatccccaggatctgcagctcgattgaccaacaagttctacgacactgatgaagaagtcgtcgcagcatgtgccgatgcgctttcccaggaatacaagatcatcaccgatgcaggtctgaccgttcagctcgacgcaccggacttggcagaagcatgggatcagatcaacccagagccaagcgtgaaggattacttagactggatcggtacacgcatcgatgccatcaacagtgcagtgaagggccttccaaaggaacagacccgcctgcacatctgctggggctcttggcacggaccacacgtcactgacatcccattcggtgacatcattggtgagatcctgcgcgcagaggtcggtggcttctccttcgaaggcgcatctcctcgtcacgcacacgagtggcgtgtatgggaagaaaacaagcttcctgaaggctctgttatctaccctggtgttgtgtctcactccatcaacgctgtggagcacccacgcctggttgctgatcgtatcgttcagttcgccaagcttgttggccctgagaacgtcattgcgtccactgactgtggtctgggcggacgtctgcattcccagatcgcatgggcaaagctggagtccctagtagagggcgctcgcattgcatcaaaggaactgttctaa

SEQ ID NO: 111 - DNA, 97 bp, Artificial Sequence
  promoter P3
tgccgtttctcgcgttgtgtgtggtactacgtggggacctaagcgtgtaagatggaaacgtctgtatcggataagtagcgaggagtgttcgttaaaa

SEQ ID NO: 112 - DNA, 35 bp, Artificial Sequence
  primer
ccaagcttgcatgcctcaccgagtctttgatcaag

SEQ ID NO: 113 - DNA, 35 bp, Artificial Sequence
  primer
caaaagttttagccacattcgggttttcaccccta

SEQ ID NO: 114 - DNA, 35 bp, Artificial Sequence
  primer
ctctggacttaaagcatgagccagaaccgcatcag

SEQ ID NO: 115 - DNA, 35 bp, Artificial Sequence
  primer
cggtacccggggatcttagaacagttcctttgatg

SEQ ID NO: 116 - DNA, 87 bp, Artificial Sequence
  DNA fragment of P8 promoter
gtggctaaaacttttggaaacttaagttacctttaatcggaaacttattgaattcgggtgaggcaactgcaactctggacttaaagc

SEQ ID NO: 117 - DNA, 35 bp, Artificial Sequence
  primer
gtgaaaacccgaatgtggctaaaacttttggaaac

SEQ ID NO: 118 - DNA, 35 bp, Artificial Sequence
  primer
gcggttctggctcatgctttaagtccagagttgca

SEQ ID NO: 119 - DNA, 1206 bp, Corynebacterium glutamicum
atgagccagaaccgcatcaggaccactcacgttggttccttgccccgtaccccagagctacttgatgcaaacatcaagcgttctaacggtgagattggggaggaggaattcttccagattctgcagtcttctgtagatgacgtgatcaagcgccaggttgacctgggtatcgacatccttaacgagggcgaatacggccacgtcacctccggtgcagttgacttcggtgcatggtggaactactccttcacccgcctgggcggactgaccatgaccgataccgaccgttgggcaagccaggaagcagtgcgttccacccctggcaacatcaagctgaccagcttctctgatcgtcgcgaccgcgcattgttcagcgaagcatacgaggatccagtatctggcatcttcaccggtcgcgcttctgtgggcaacccagagttcaccggacctattacctacattggccaggaagaaactcagacggatgttgatctgctgaagaagggcatgaacgcagcgggagctaccgacggcttcgttgcagcactatccccaggatctgcagctcgattgaccaacaagttctacgacactgatgaagaagtcgtcgcagcatgtgctgatgcgctttcccaggaatacaagatcatcaccgatgcaggtctgaccgttcagctcgacgcaccggacttggcagaagcatgggatcagatcaacccagagccaagcgtgaaggattacttggactggatcggtacacgcatcgatgccatcaacagtgcagtgaagggccttccaaaggaacagacccgcctgcacatctgctggggctcttggcacggaccacacgtcactgacatcccattcggtgacatcattggtgagatcctgcgcgcagaggtcggtggcttctccttcgaaggcgcatctcctcgtcacgcacacgagtggcgtgtatgggaagaaaacaagcttcctgaaggctctgttatctaccctggtgttgtgtctcactccatcaacgctgtggagcacccacgcctggttgctgatcgtatcgttcagttcgccaagcttgttggccctgagaacgtcattgcgtccactgactgtggtctgggcggacgtctgcattcccagatcgcatgggcaaagctggagtccctagtagagggcgctcgcattgcatcaaaggaactgttctaa

SEQ ID NO: 120 - protein, 401 aa, Corynebacterium glutamicum
MSQNRIRTTHVGSLPRTPELLDANIKRSNGEIGEEEFFQILQSSVDDVIKRQVDLGIDILNEGEYGHVTSGAVDFGAWWNYSFTRLGGLTMTDTDRWASQEAVRSTPGNIKLTSFSDRRDRALFSEAYEDPVSGIFTGRASVGNPEFTGPITYIGQEETQTDVDLLKKGMNAAGATDGFVAALSPGSAARLTNKFYDTDEEVVAACADALSQEYKIITDAGLTVQLDAPDLAEAWDQINPEPSVKDYLDWIGTRIDAINSAVKGLPKEQTRLHICWGSWHGPHVTDIPFGDIIGEILRAEVGGFSFEGASPRHAHEWRVWEENKLPEGSVIYPGVVSHSINAVEHPRLVADRIVQFAKLVGPENVIASTDCGLGGRLHSQIAWAKLESLVEGARIASKELF

SEQ ID NO: 121 - DNA, 35 bp, Artificial Sequence
  primer
ccaagcttgcatgccccctcatgagttcaggggtt

SEQ ID NO: 122 - DNA, 35 bp, Artificial Sequence
  primer
tggtataaatttattaaactacccatatccccagc

SEQ ID NO: 123 - DNA, 35 bp, Artificial Sequence
  primer
cttaaggacctccaagtggctgaaatcatgcacgt

SEQ ID NO: 124 - DNA, 35 bp, Artificial Sequence
  primer
cggtacccggggatcttagccctgaaagcgtggga

SEQ ID NO: 125 - DNA, 98 bp, Artificial Sequence
  DNA fragment of P4 promoter
aataaatttataccacacagtctattgcaatagaccaagctgttcagtagggtgcatgggagaagaatttcctaataaaaactcttaaggacctccaa

SEQ ID NO: 126 - DNA, 35 bp, Artificial Sequence
  primer
ggatatgggtagtttaataaatttataccacacag

SEQ ID NO: 127 - DNA, 35 bp, Artificial Sequence
  primer
catgatttcagccacttggaggtccttaagagttt

SEQ ID NO: 128 - DNA, 1278 bp, Corynebacterium glutamicum
gtggctgaaatcatgcacgtattcgctcgcgaaattctcgactcccgcggtaacccaaccgtcgaggcagaggttttccttgatgacggttcccacggtgtcgcaggtgttccatccggcgcatccaccggcgtccacgaggctcatgagctgcgtgacggtggcgatcgctacctgggcaagggcgttttgaaggcagttgaaaacgtcaacgaagaaatcggcgacgagctcgctggcctagaggctgacgatcagcgcctcatcgacgaagcaatgatcaagcttgatggcaccgccaacaagtcccgcctgggtgcaaacgcaatccttggtgtttccatggctgttgcaaaggctgctgctgattccgcaggcctcccactgttccgctacatcggtggaccaaacgcacacgttcttccagttccaatgatgaacatcatcaacggtggcgctcacgctgactccggtgttgacgttcaggaattcatgatcgctccaatcggtgcagagaccttctctgaggctctccgcaacggcgcagaggtctaccacgcactgaagtccgtcatcaaggaaaagggcctgtccaccggacttggcgatgagggcggcttcgctccttccgtcggctccacccgtgaggctcttgaccttatcgttgaggcaatcgagaaggctggcttcaccccaggcaaggacatcgctcttgctctggacgttgcttcctctgagttcttcaaggacggcacctaccacttcgaaggtggccagcactccgcagctgagatggcaaacgtttacgctgagctcgttgacgcgtacccaatcgtctccatcgaggacccactgcaggaagatgactgggagggttacaccaacctcaccgcaaccatcggcgacaaggttcagatcgttggcgacgacttcttcgtcaccaaccctgagcgcctgaaggagggcatcgctaagaaggctgccaactccatcctggttaaggtgaaccagatcggtaccctcaccgagaccttcgacgctgtcgacatggctcaccgcgcaggctacacctccatgatgtcccaccgttccggtgagaccgaggacaccaccattgctgacctcgcagttgcactcaactgtggccagatcaagactggtgctccagcacgttccgaccgtgtcgcaaagtacaaccagcttctccgcatcgagcagttgcttggcgacgccggcgtctacgcaggtcgcagcgcattcccacgctttcagggctaa

SEQ ID NO: 129 - protein, 425 aa, Corynebacterium glutamicum
MAEIMHVFAREILDSRGNPTVEAEVFLDDGSHGVAGVPSGASTGVHEAHELRDGGDRYLGKGVLKAVENVNEEIGDELAGLEADDQRLIDEAMIKLDGTANKSRLGANAILGVSMAVAKAAADSAGLPLFRYIGGPNAHVLPVPMMNIINGGAHADSGVDVQEFMIAPIGAETFSEALRNGAEVYHALKSVIKEKGLSTGLGDEGGFAPSVGSTREALDLIVEAIEKAGFTPGKDIALALDVASSEFFKDGTYHFEGGQHSAAEMANVYAELVDAYPIVSIEDPLQEDDWEGYTNLTATIGDKVQIVGDDFFVTNPERLKEGIAKKAANSILVKVNQIGTLTETFDAVDMAHRAGYTSMMSHRSGETEDTTIADLAVALNCGQIKTGAPARSDRVAKYNQLLRIEQLLGDAGVYAGRSAFPRFQG

SEQ ID NO: 130 - DNA, 666 bp, Homo sapiens
atgggtgacaccaaggagcagcgcatcctgaaccacgtgctgcagcatgcggagcccgggaacgcacagagcgtgctggaggccattgacacctactgcgagcagaaggagtgggccatgaacgtgggcgacaagaaaggcaagatcgtggacgccgtgattcaggagcaccagccctccgtgctgctggagctgggggcctactgtggctactcagctgtgcgcatggcccgcctgctgtcaccaggggcgaggctcatcaccatcgagatcaaccccgactgtgccgccatcacccagcggatggtggatttcgctggcgtgaaggacaaggtcacccttgtggttggagcgtcccaggacatcatcccccagctgaagaagaagtatgatgtggacacactggacatggtcttcctcgaccactggaaggaccggtacctgccggacacgcttctcttggaggaatgtggcctgctgcggaaggggacagtgctactggctgacaacgtgatctgcccaggtgcgccagacttcctagcacacgtgcgcgggagcagctgctttgagtgcacacactaccaatcgttcctggaatacagggaggtggtggacggcctggagaaggccatctacaagggcccaggcagcgaagcagggccttaa

SEQ ID NO: 131 - DNA, 675 bp, Homo sapiens
catatgggggataccaaagaacagcggattctgaatcatgttttacagcacgctgaaccgggcaatgctcagagcgttttagaagcaatagatacctattgtgaacagaaggaatgggcaatgaatgttggcgataaaaagggcaaaattgttgatgcagttatccaggaacatcagccgagcgttttacttgaactgggcgcatattgcggttattccgcagttcggatggcacggctgctgtcccctggcgctcgcttaattaccattgaaattaatccggattgcgcagcaattacccagcggatggttgactttgcaggtgttaaagataaagtcaccttggttgtcggcgctagccaggatattattccgcagctgaaaaaaaaatacgatgttgataccctggatatggtctttttagatcattggaaagatcggtatctgcccgatactctgttattggaagagtgcggtctgctgcggaaaggcaccgttctactggcagataatgttatttgtcctggggctcctgattttctagctcatgttcggggcagcagctgtttcgaatgtacccattaccaatcgtttctggaatatcgcgaagttgttgatggtctggaaaaggcaatttataaaggtcctggtagcgaggctggcccgtaagagctc

SEQ ID NO: 132 - DNA, 6557 bp, Artificial Sequence
  pELAC vector
tggcgaatgggacgcgccctgtagcggcgcattaagcgcggcgggtgtggtggttacgcgcagcgtgaccgctacacttgccagcgccctagcgcccgctcctttcgctttcttcccttcctttctcgccacgttcgccggctttccccgtcaagctctaaatcgggggctccctttagggttccgatttagtgctttacggcacctcgaccccaaaaaacttgattagggtgatggttcacgtagtgggccatcgccctgatagacggtttttcgccctttgacgttggagtccacgttctttaatagtggactcttgttccaaactggaacaacactcaaccctatctcggtctattcttttgatttataagggattttgccgatttcggcctattggttaaaaaatgagctgatttaacaaaaatttaacgcgaattttaacaaaatattaacgtttacaatttcaggtggcacttttcggggaaatgtgcgcggaacccctatttgtttatttttctaaatacattcaaatatgtatccgctcatgagacaataaccctgataaatgcttcaataatattgaaaaaggaagagtatgagtattcaacatttccgtgtcgcccttattcccttttttgcggcattttgccttcctgtttttgctcacccagaaacgctggtgaaagtaaaagatgctgaagatcagttgggtgcacgagtgggttacatcgaactggatctcaacagcggtaagatccttgagagttttcgccccgaagaacgttttccaatgatgagcacttttaaagttctgctatgtggcgcggtattatcccgtattgacgccgggcaagagcaactcggtcgccgcatacactattctcagaatgacttggttgagtactcaccagtcacagaaaagcatcttacggatggcatgacagtaagagaattatgcagtgctgccataaccatgagtgataacactgcggccaacttacttctgacaacgatcggaggaccgaaggagctaaccgcttttttgcacaacatgggggatcatgtaactcgccttgatcgttgggaaccggagctgaatgaagccataccaaacgacgagcgtgacaccacgatgcctgcagcaatggcaacaacgttgcgcaaactattaactggcgaactacttactctagcttcccggcaacaattaatagactggatggaggcggataaagttgcaggaccacttctgcgctcggcccttccggctggctggtttattgctgataaatctggagccggtgagcgtgggtctcgcggtatcattgcagcactggggccagatggtaagccctcccgtatcgtagttatctacacgacggggagtcaggcaactatggatgaacgaaatagacagatcgctgagataggtgcctcactgattaagcattggtaactgtcagaccaagtttactcatatatactttagattgatttaaaacttcatttttaatttaaaaggatctaggtgaagatcctttttgataatctcatgaccaaaatcccttaacgtgagttttcgttccactgagcgtcagaccccgtagaaaagatcaaaggatcttcttgagatcctttttttctgcgcgtaatctgctgcttgcaaacaaaaaaaccaccgctaccagcggtggtttgtttgccggatcaagagctaccaactctttttccgaaggtaactggcttcagcagagcgcagataccaaatactgtccttctagtgtagccgtagttaggccaccacttcaagaactctgtagcaccgcctacatacctcgctctgctaatcctgttaccagtggctgctgccagtggcgataagtcgtgtcttaccgggttggactcaagacgatagttaccggataaggcgcagcggtcgggctgaacggggggttcgtgcacacagcccagcttggagcgaacgacctacaccgaactgagatacctacagcgtgagctatgagaaagcgccacgcttcccgaagggagaaaggcggacaggtatccggtaagcggcagggtcggaacaggagagcgcacgagggagcttccagggggaaacgcctggtatctttatagtcctgtcgggtttcgccacctctgacttgagcgtcgatttttgtgatgctcgtcaggggggcggagcctatggaaaaacgccagcaacgcggcctttttacggttcctggccttttgctggccttttgctcacatgttctttcctgcgttatcccctgattctgtggataaccgtattaccgcctttgagtgagctgataccgctcgccgcagccgaacgaccgagcgcagcgagtcagtgagcgaggaagcggaagagcgcctgatgcggtattttctccttacgcatctgtgcggtatttcacaccgcatatatggtgcactctcagtacaatctgctctgatgccgcatagttaagccagtatacactccgctatcgctacgtgactgggtcatggctgcgccccgacacccgccaacacccgctgacgcgccctgacgggcttgtctgctcccggcatccgcttacagacaagctgtgaccgtctccgggagctgcatgtgtcagaggttttcaccgtcatcaccgaaacgcgcgaggcagctgcggtaaagctcatcagcgtggtcgtgaagcgattcacagatgtctgcctgttcatccgcgtccagctcgttgagtttctccagaagcgttaatgtctggcttctgataaagcgggccatgttaagggcggttttttcctgtttggtcactgatgcctccgtgtaagggggatttctgttcatgggggtaatgataccgatgaaacgagagaggatgctcacgatacgggttactgatgatgaacatgcccggttactggaacgttgtgagggtaaacaactggcggtatggatgcggcgggaccagagaaaaatcactcagggtcaatgccagcgcttcgttaatacagatgtaggtgttccacagggtagccagcagcatcctgcgatgcagatccggaacataatggtgcagggcgctgacttccgcgtttccagactttacgaaacacggaaaccgaagaccattcatgttgttgctcaggtcgcagacgttttgcagcagcagtcgcttcacgttcgctcgcgtatcggtgattcattctgctaaccagtaaggcaaccccgccagcctagccgggtcctcaacgacaggagcacgatcatgcgcacccgtggggccgccatgccggcgataatggcctgcttctcgccgaaacgtttggtggcgggaccagtgacgaaggcttgagcgagggcgtgcaagattccgaataccgcaagcgacaggccgatcatcgtcgcgctccagcgaaagcggtcctcgccgaaaatgacccagagcgctgccggcacctgtcctacgagttgcatgataaagaagacagtcataagtgcggcgacgatagtcatgccccgcgcccaccggaaggagctgactgggttgaaggctctcaagggcatcggtcgagatcccggtgcctaatgagtgagctaacttacattaattgcgttgcgctcactgcccgctttccagtcgggaaacctgtcgtgccagctgcattaatgaatcggccaacgcgcggggagaggcggtttgcgtattgggcgccagggtggtttttcttttcaccagtgagacgggcaacagctgattgcccttcaccgcctggccctgagagagttgcagcaagcggtccacgctggtttgccccagcaggcgaaaatcctgtttgatggtggttaacggcgggatataacatgagctgtcttcggtatcgtcgtatcccactaccgagatatccgcaccaacgcgcagcccggactcggtaatggcgcgcattgcgcccagcgccatctgatcgttggcaaccagcatcgcagtgggaacgatgccctcattcagcatttgcatggtttgttgaaaaccggacatggcactccagtcgccttcccgttccgctatcggctgaatttgattgcgagtgagatatttatgccagccagccagacgcagacgcgccgagacagaacttaatgggcccgctaacagcgcgatttgctggtgacccaatgcgaccagatgctccacgcccagtcgcgtaccgtcttcatgggagaaaataatactgttgatgggtgtctggtcagagacatcaagaaataacgccggaacattagtgcaggcagcttccacagcaatggcatcctggtcatccagcggatagttaatgatcagcccactgacgcgttgcgcgagaagattgtgcaccgccgctttacaggcttcgacgccgcttcgttctaccatcgacaccaccacgctggcacccagttgatcggcgcgagatttaatcgccgcgacaatttgcgacggcgcgtgcagggccagactggaggtggcaacgccaatcagcaacgactgtttgcccgccagttgttgtgccacgcggttgggaatgtaattcagctccgccatcgccgcttccactttttcccgcgttttcgcagaaacgtggctggcctggttcaccacgcgggaaacggtctgataagagacaccggcatactctgcgacatcgtataacgttactggtttcacattcaccaccctgaattgactctcttccgggcgctatcatgccataccgcgaaaggttttgcgccattcgatggtgtccgggatctcgacgctctcccttatgcgactcctgcattaggaagcagcccagtagtaggttgaggccgttgagcaccgccgccgcaaggaatggtgcatgcaaggagatggcgcccaacagtcccccggccacggggcctgccaccatacccacgccgaaacaagcgctcatgagcccgaagtggcgagcccgatcttccccatcggtgatgtcggcgatataggcgccagcaaccgcacctgtggcgccggtgatgccggccacgatgcgtccggcgtagaggatcgagatctgcgggcagtgagcgcaacgcaattaatgtgagttagctcactcattaggcaccccaggctttacactttatgcttccggctcgtataatgtgtggaattgtgagcggataacaatttcacacaggatctagatttaagaaggagatatacatatggccgaagaaggtaaactggtaatctggattaacggcgataaaggctataacggtctcgctgaagtcggtaagaaattcgagaaagataccggaattaaagtcaccgttgagcatccggataaactggaagagaaattcccacaggttgcggcaacaggcgatggccctgacattatcttctgggcacacgaccgctttggtggctacgctcaatctggcctgttggctgaaatcaccccggacaaagcgttccaggacaagctgtatccgtttacctgggatgccgtacgttacaacggcaagctgattgcttacccgatcgctgttgaagcgttatcgctgatttataacaaagatctgctgccgaacccgccaaaaacctgggaagagatcccggcgctggataaagaactgaaagcgaaaggtaagagcgcgctgatgttcaacctgcaagaaccgtacttcacctggccgctgattgctgctgacgggggttatgcgttcaagtatgaaaacggcaagtacgacattaaagacgtgggcgtggataacgctggcgcgaaagcgggtctgaccttcctggttgacctgattaaaaacaaacacatgaatgcagacaccgattactccatcgcagaagctgcctttaataaaggcgaaacagcgatgaccatcaacggcccgtgggcatggtccaacatcgacaccagcaaagtgaattatggtgtaacggtactgccgaccttcaagggtcaaccatccaaaccgttcgttggcgtgctgagcgcaggtattaacgccgccagtccgaacaaagagctggcaaaagagttcctcgaaaactatctgctgactgatgaaggtctggaagcggttaataaagacaaaccgctgggtgccgtagcgctgaagtcttacgaggaagagttggcgaaagatccacgtattgccgccactatggaaaacgcccagaaaggtgaaatcatgccgaacatcccgcagatgtccgctttctggtatgccgtgcgtactgcggtgatcaacgccgccagcggtcgtcagactgtcgatgaagccctgaaagacgcgcagactaaggatccgaattcgagctccgtcgacaagcttgcggccgcactcgagcaccaccaccaccaccactgagatccggctgctaacaaagcccgaaaggaagctgagttggctgctgccaccgctgagcaataactagcataaccccttggggcctctaaacgggtcttgaggggttttttgctgaaaggaggaactatatccggat

SEQ ID NO: 133 - DNA, 22 bp, Artificial Sequence
  primer
gtgagttagctcactcattagg

SEQ ID NO: 134 - DNA, 22 bp, Artificial Sequence
  primer
cgattggtaatgggtacattcg

SEQ ID NO: 135 - DNA, 20 bp, Artificial Sequence
  primer
ggatctcagtggtggtggtg

SEQ ID NO: 136 - DNA, 44 bp, Artificial Sequence
  primer
ccaagcttgcatgccaaattcctgtgaattagctgatttagtac

SEQ ID NO: 137 - DNA, 38 bp, Artificial Sequence
  primer
tttggtatcccccatagaggcgaaggctccttgaatag

SEQ ID NO: 138 - DNA, 22 bp, Artificial Sequence
  primer
atgggggataccaaagaacagc

SEQ ID NO: 139 - DNA, 38 bp, Artificial Sequence
  primer
cggtacccggggatcatgctagttattgctcagcggtg

SEQ ID NO: 140 - DNA, 666 bp, Niastella koreensis
atgaataatcaaatttttgaatccgttgaccattatatcagcgatttactgggttacgaagacgatgcattgcttgccgccaccaattcattagccgaagcaggcatgcctgccatcagcgtatcacccaaccagggcaagtttctgcaattactggcccaattgtgccaggcaaaaaatatcctggagctgggcacactggcaggctacagcaccatttggatggcccgggccttacccaaaaacggccggctcatcacccttgaatatgaccccaaacatgcggccgttgcacaaaaaaatatcgaccgggccggccttacttcacaagtacagatcagaaccggtaaagcaattgacatattaccgcaattagtggaagaaggcgccggaccttttgatatgatctttatcgatgccgataaaccaccttacaccgaatattttcaatgggcgcttcggttatcacgtcccggtacactcatcgtggccgataatgtgatccgtgatggcaaagtgctggatgaaaacagtacggagcctgctgtacagggcgcaagacgtttcaatgccatgctgggcgccaataccgccgttgacgccaccattcttcaaatggtaggtgtaaaagaatacgatggaatggctttggccatagtaaaataa

SEQ ID NO: 141 - protein, 221 aa, Niastella koreensis
MNNQIFESVDHYISDLLGYEDDALLAATNSLAEAGMPAISVSPNQGKFLQLLAQLCQAKNILELGTLAGYSTIWMARALPKNGRLITLEYDPKHAAVAQKNIDRAGLTSQVQIRTGKAIDILPQLVEEGAGPFDMIFIDADKPPYTEYFQWALRLSRPGTLIVADNVIRDGKVLDENSTEPAVQGARRFNAMLGANTAVDATILQMVGVKEYDGMALAIVK

SEQ ID NO: 142 - DNA, 50 bp, Artificial Sequence
  primer
catgattacgccaagcttgcatgccaaattcctgtgattagctgatttag

SEQ ID NO: 143 - DNA, 50 bp, Artificial Sequence
  primer
cggattcgaagatctggttgttcatagaggcgaaggctccttgaataggt

SEQ ID NO: 144 - DNA, 778 bp, Niastella koreensis
atgaacaaccagatcttcgaatccgtcgatcactatatttctgatcttctgggctacgaggatgatgcgcttttggccgccactaattccctggccgaggcaggtatgccggctattagcgtttccccgaaccagggcaaatttttgcaactgctggcccaactttgccaagccaaaaacattttggagcttggtacgttggccggctattcgaccatctggatggctcgcgctctccccaagaacggccgccttatcaccctggaatacgatccgaagcatgccgcggtagctcagaagaacattgatcgcgctggcttgaccagccaagtgcaaatccgcacgggtaaagcaatcgacatcctgccgcagctggtggaggagggtgccggtccatttgatatgatcttcattgatgccgataagcccccatacaccgaatactttcaatgggctctgcgactgtcccgccccggcactctcatcgtcgcggataatgtcatccgcgatggaaaggtgctggacgaaaactccaccgagcctgccgtccaaggtgcccgccgttttaatgccatgctcggtgctaatacggcagttgacgcaaccatcctccaaatggtgggcgtgaaagagtacgacggcatggcgctggccatcgttaagtaaaagcttgcggccgcactcgagcaccaccaccaccaccactgagatccggctgctaacaaagcccgaaaggaagctgagttggctgctgccaccgctgagcaataactagcat

SEQ ID NO: 145 - DNA, 666 bp, Niastella koreensis
atgaacaaccagatcttcgaatccgtcgatcactatatttctgatcttctgggctacgaggatgatgcgcttttggccgccactaattccctggccgaggcaggtatgccggctattagcgtttccccgaaccagggcaaatttttgcaactgctggcccaactttgccaagccaaaaacattttggagcttggtacgttggccggctattcgaccatctggatggctcgcgctctccccaagaacggccgccttatcaccctggaatacgatccgaagcatgccgcggtagctcagaagaacattgatcgcgctggcttgaccagccaagtgcaaatccgcacgggtaaagcaatcgacatcctgccgcagctggtggaggagggtgccggtccatttgatatgatcttcattgatgccgataagcccccatacaccgaatactttcaatgggctctgcgactgtcccgccccggcactctcatcgtcgcggataatgtcatccgcgatggaaaggtgctggacgaaaactccaccgagcctgccgtccaaggtgcccgccgttttaatgccatgctcggtgctaatacggcagttgacgcaaccatcctccaaatggtgggcgtgaaagagtacgacggcatggcgctggccatcgttaagtaa

SEQ ID NO: 146 - DNA, 33 bp, Artificial Sequence
  primer
ctggccgaggcaggtaagccggctattagcgtt

SEQ ID NO: 147 - DNA, 33 bp, Artificial Sequence
  primer
aacgctaatagccggcttacctgcctcggccag

SEQ ID NO: 148 - DNA, 33 bp, Artificial Sequence
  primer
ctggccgaggcaggtgttccggctattagcgtt

SEQ ID NO: 149 - DNA, 33 bp, Artificial Sequence
  primer
aacgctaatagccggaacacctgcctcggccag

SEQ ID NO: 150 - DNA, 33 bp, Artificial Sequence
  primer
cttatcaccctggaatgtgatccgaagcatgcc

SEQ ID NO: 151 - DNA, 33 bp, Artificial Sequence
  primer
ggcatgcttcggatcacattccagggtgataag

SEQ ID NO: 152 - DNA, 33 bp, Artificial Sequence
  primer
cttatcaccctggaaggggatccgaagcatgcc

SEQ ID NO: 153 - DNA, 33 bp, Artificial Sequence
  primer
ggcatgcttcggatccccttccagggtgataag

SEQ ID NO: 154 - DNA, 33 bp, Artificial Sequence
  primer
cttatcaccctggaaagtgatccgaagcatgcc

SEQ ID NO: 155 - DNA, 33 bp, Artificial Sequence
  primer
ggcatgcttcggatcactttccagggtgataag

SEQ ID NO: 156 - DNA, 33 bp, Artificial Sequence
  primer
gatgccgataagcccggttacaccgaatacttt

SEQ ID NO: 157 - DNA, 33 bp, Artificial Sequence
  primer
aaagtattcggtgtaaccgggcttatcggcatc

SEQ ID NO: 158 - DNA, 33 bp, Artificial Sequence
  primer
gatgccgataagccctcttacaccgaatacttt

SEQ ID NO: 159 - DNA, 33 bp, Artificial Sequence
  primer
aaagtattcggtgtaagagggcttatcggcatc

SEQ ID NO: 160 - DNA, 33 bp, Artificial Sequence
  primer
gatgccgataagcccagttacaccgaatacttt

SEQ ID NO: 161 - DNA, 33 bp, Artificial Sequence
  primer
aaagtattcggtgtaactgggcttatcggcatc

SEQ ID NO: 162 - DNA, 33 bp, Artificial Sequence
  primer
gatgccgataagcccgtgtacaccgaatacttt

SEQ ID NO: 163 - DNA, 33 bp, Artificial Sequence
  primer
aaagtattcggtgtacacgggcttatcggcatc

SEQ ID NO: 164 - DNA, 33 bp, Artificial Sequence
  primer
gatgccgataagccctattacaccgaatacttt

SEQ ID NO: 165 - DNA, 33 bp, Artificial Sequence
  primer
aaagtattcggtgtaatagggcttatcggcatc

SEQ ID NO: 166 - DNA, 7651 bp, Artificial Sequence
  common part of some pVK9-based expression plasmids
cgcagcaggcatgagcagcccgaatatgcgcctgctggctgcaacgaccgaggaaatgacccgcgttttcggcgctgaccaggctttttcacataggctgagccggtggccactgcacgtctccgacgatcccaccgcgtaccgctggcatgcccagcacaatcgcgtggatcgcctagctgatcccgaaaaagtttttgccttttgtaaaaaacttctcggtcgccccgcaaattttcgattccagattttttaaaaaccaagccagaaatacgacacaccgtttgcagataatctgtctttcggaaaaatcaagtgcgatacaaaatttttagcacccctgagctgcgcaaagtcccgcttcgtgaaaattttcgtgccgcgtgattttccgccaaaaactttaacgaacgttcgttataatggtgtcatgaccttcacgacgaagtaccaaaattggcccgaatcatcagctatggatctctctgatgtcgcgctggagtccgacgcgctcgatgctgccgtcgatttaaaaacggtgatcggatttttccgagctctcgatacgacggacgcgccagcatcacgagactgggccagtgccgcgagcgacctagaaactctcgtggcggatcttgaggagctggctgacgagctgcgtgctcggcagcgccaggaggacgcacagtagtggaggatcgaatcagttgcgcctactgcggtggcctgattcctccccggcctgacccgcgaggacggcgcgcaaaatattgctcagatgcgtgtcgtgccgcagccagccgcgagcgcgccaacaaacgccacgccgaggagctggaggcggctaggtcgcaaatggcgctggaagtgcgtcccccgagcgaaattttggccatggtcgtcacagagctggaagcggcagcgagaattatccgcgatcgtggcgcggtgcccgcaggcatgacaaacatcgtaaatgccgcgtttcgtgtggccgtggccgcccaggacgtgtcagcgccgccaccacctgcaccgaatcggcagcagcgtcgcgcgtcgaaaaagcgcacaggcggcaagaagcgataagctgcacgaatacctgaaaaatgttgaacgccccgtgagcggtaactcacagggcgtcggctaacccccagtccaaacctgggagaaagcgctcaaaaatgactctagcggattcacgagacattgacacaccggcctggaaattttccgctgatctgttcgacacccatcccgagctcgcgctgcgatcacgtggctggacgagcgaagaccgccgcgaattcctcgctcacctgggcagagaaaatttccagggcagcaagacccgcgacttcgccagcgcttggatcaaagacccggacacgggagaaacacagccgaagttataccgagttggttcaaaatcgcttgcccggtgccagtatgttgctctgacgcacgcgcagcacgcagccgtgcttgtcctggacattgatgtgccgagccaccaggccggcgggaaaatcgagcacgtaaaccccgaggtctacgcgattttggagcgctgggcacgcctggaaaaagcgccagcttggatcggcgtgaatccactgagcgggaaatgccagctcatctggctcattgatccggtgtatgccgcagcaggcatgagcagcccgaatatgcgcctgctggctgcaacgaccgaggaaatgacccgcgttttcggcgctgaccaggctttttcacataggctgagccggtggccactgcacgtctccgacgatcccaccgcgtaccgctggcatgcccagcacaatcgcgtggatcgcctagctgatcttatggaggttgctcgcatgatctcaggcacagaaaaacctaaaaaacgctatgagcaggagttttctagcggacgggcacgtatcgaagcggcaagaaaagccactgcggaagcaaaagcacttgccacgcttgaagcaagcctgccgagcgccgctgaagcgtctggagagctgatcgacggcgtccgtgtcctctggactgctccagggcgtgccgcccgtgatgagacggcttttcgccacgctttgactgtgggataccagttaaaagcggctggtgagcgcctaaaagacaccaagatcatcgacgcctacgagcgtgcctacaccgtcgctcaggcggtcggagcagacggccgtgagcctgatctgccgccgatgcgtgaccgccagacgatggcgcgacgtgtgcgcggctacgtcgctaaaggccagccagtcgtccctgctcgtcagacagagacgcagagcagccgagggcgaaaagctctggccactatgggaagacgtggcggtaaaaaggccgcagaacgctggaaagacccaaacagtgagtacgcccgagcacagcgagaaaaactagctaagtccagtcaacgacaagctaggaaagctaaaggaaatcgcttgaccattgcaggttggtttatgactgttgagggagagactggctcgtggccgacaatcaatgaagctatgtctgaatttagcgtgtcacgtcagaccgtgaatagagcacttaagtctgcgggcattgaacttccacgaggacgccgtaaagcttcccagtaaatgtgccatctcgtaggcagaaaacggttccccccgtaggggtctctctcttggcctcctttctaggtcgggctgattgctcttgaagctctctaggggggctcacaccataggcagataacggttccccaccggctcacctcgtaagcgcacaaggactgctcccaaagatcgcctagctgatcttatggaggttgctcgcatgatcctttttgataatctcatgaccaaaatcccttaacgtgagttttcgttccactgagcgtcagaccccgtagaaaagatccccgtccacctacaacaaagctctcatcaaccgtggctccctcactttctggctggatgatggggcgattcaggcctggtatgagtcagcaacaccttcttcacgaggcagacctctcgacggagttccactgagcgtcagaccccgtagaaaagatcaaaggatcttcttgagatcctttttttctgcgcgtaatctgctgcttgcaaacaaaaaaaccaccgctaccagcggtggtttgtttgccggatcaagagctaccaactctttttccgaaggtaactggcttcagcagagcgcagataccaaatactgttcttctagtgtagccgtagttaggccaccacttcaagaactctgtagcaccgcctacatacctcgctctgctaatcctgttaccagtggctgctgccagtggcgataagtcgtgtcttaccgggttggactcaagacgatagttaccggataaggcgcagcggtcgggctgaacggggggttcgtgcacacagcccagcttggagcgaacgacctacaccgaactgagatacctacagcgtgagctatgagaaagcgccacgcttcccgaagggagaaaggcggacaggtatccggtaagcggcagggtcggaacaggagagcgcacgagggagcttccagggggaaacgcctggtatctttatagtcctgtcgggtttcgccacctctgacttgagcgtcgatttttgtgatgctcgtcaggggggcggagcctatggaaaaacgccagcaacgcggcctttttacggttcctggccttttgctggccttttgctcacatgttctttcctgcgttatcccctgattctgtggataaccgtattaccgcctttgagtgagctgataccgctcgccgcagccgaacgaccgagcgcagcgagtcagtgagcgaggaagcggaagaagctcgcacattcagcagcgtttttcagcgcgttttcgatcaacgtttcaatgttggtatcaacaccaggtttaactttgaacttatcggcactgacggttactgattttgaacttttgctttgccacggaacggtctgcgttgtcgggaagatgcgtgatctgatccttcaactcagcaaaagttcccaatacgcaaaccgcctctccccgcgcgttggccgattcattaatgcagctggcacgacaggtttcccgactggaaagcgggcagtgagcgcaacgcaattaatgtgagttagctcactcattaggcaccccaggctttacactttatgcttccggctcgtatgttgtgtggaattgtgagcggataacaatttcacacaggaaacagctatgaccatgattacgccaagcttgcatgccaaattcctgtgattagctgatttagtacttttcggaggtgtctattcttaccaaatcgtcaagttgtgggtagagtcacctgaatattaattgcaccgcacgggtgatatatgcttatttgctcaagtagttcgaggttaagtgtattttaggtgaacaaatttcagcttcgggtagaagactttcgatgcgcttcagagcttctattgggaaatctgacaccacttgattaaatagcctacccccgaattgggggattggtcattttttgctgtgaaggtagttttgatgcatatgacctgcgtttataaagaaatgtaaacgtgatcagatcgatataaaagaaacagtttgtactcaggtttgaagcattttctccgattcgcctggcaaaaatctcaattgtcgcttacagtttttctcaacgacaggctgctaagctgctagttcggtggcctagtgagtggcgtttacttggataaaagtaatcccatgtcgtgatcagccattttgggttgtttccatagcaatccaaaggtttcgtctttcgatacctattcaaggagccttcgcctctgagctccgtcgacaagcttgcggccgcactcgagcaccaccaccaccaccactgagatccggctgctaacaaagcccgaaaggaagctgagttggctgctgccaccgctgagcaataactagcatgatccccgggtaccgagctcgaattcactggccgtcgttttacaacgtcgtgactgggaaaaccctggcgttacccaacttaatcgccttgcagcacatccccctttcgccagctggcgtaatagcgaagaggcccgcaccgatcgcccttcccaacagttgcgcagcctgaatggcgaatgcgatttattcaacaaagccgccgtcccgtcaagtcagcgtaatgctctgccctgatgaatcccctaatgattttggtaaaaatcattaagttaaggtggatacacatcttgtcatatgatcaaatggtttcgcgaaaaatcaataatcagacaacaagatgtgcgaactcgatattttacacgactctctttaccaattctgccccgaattacacttaaaacgactcaacagcttaacgttggcttgccacgcattacttgactgtaaaactctcactcttaccgaacttggccgtaacctgccaaccaaagcgagaacaaaacataacatcaaacgaatcgaccgattgttaggtaatcgtcacctccacaaagagcgactcgctgtataccgttggcatgctagctttatctgttcgggcaatacgatgcccattgtacttgttgactggtctgatattcgtgagcaaaaacgacttatggtattgcgagcttcagtcgcactacacggtcgttctgttactctttatgagaaagcgttcccgctttcagagcaatgttcaaagaaagctcatgaccaatttctagccgaccttgcgagcattctaccgagtaacaccacaccgctcattgtcagtgatgctggctttaaagtgccatggtataaatccgttgagaagctgggttggtactggttaagtcgagtaagaggaaaagtacaatatgcagacctaggagcggaaaactggaaacctatcagcaacttacatgatatgtcatctagtcactcaaagactttaggctataagaggctgactaaaagcaatccaatctcatgccaaattctattgtataaatctcgctctaaaggccgaaaaaatcagcgctcgacacggactcattgtcaccacccgtcacctaaaatctactcagcgtcggcaaaggagccatgggttctagcaactaacttacctgttgaaattcgaacacccaaacaacttgttaatatctattcgaagcgaatgcagattgaagaaaccttccgagacttgaaaagtcctgcctacggactaggcctacgccatagccgaacgagcagctcagagcgttttgatatcatgctgctaatcgccctgatgcttcaactaacatgttggcttgcgggcgttcatgctcagaaacaaggttgggacaagcacttccaggctaacacagtcagaaatcgaaacgtactctcaacagttcgcttaggcatggaagttttgcggcattctggctacacaataacaagggaagacttactcgtggctgcaaccctactagctcaaaatttattcacacatggttacgctttggggaaattatgaggggatctctcagtgctctgccagtgttacaaccaattaaccaattctgattagaaaaactcatcgagcatcaaatgaaactgcaatttattcatatcaggattatcaataccatatttttgaaaaagccgtttctgtaatgaaggagaaaactcaccgaggcagttccataggatggcaagatcctggtatcggtctgcgattccgactcgtccaacatcaatacaacctattaatttcccctcgtcaaaaataaggttatcaagtgagaaatcaccatgagtgacgactgaatccggtgagaatggcaaaagcttatgcatttctttccagacttgttcaacaggccagccattacgctcgtcatcaaaatcactcgcatcaaccaaaccgttattcattcgtgattgcgcctgagcgagacgaaatacgcgatcgctgttaaaaggacaattacaaacaggaatcgaatgcaaccggcgcaggaacactgccagcgcatcaacaatattttcacctgaatcaggatattcttctaatacctggaatgctgttttcccggggatcgcagtggtgagtaaccatgcatcatcaggagtacggataaaatgcttgatggtcggaagaggcataaattccgtcagccagtttagtctgaccatctcatctgtaacatcattggcaacgctacctttgccatgtttcagaaacaactctggcgcatcgggcttcccatacaatcgatagattgtcgcacctgattgcccgacattatcgcgagcccatttatacccatataaatcagcatccatgttggaatttaatcgcggcttcgagcaagacgtttcccgttgaatatggctcataacaccccttgtattactgtttatgtaagcagacagttttattgttcatgatgatatatttttatcttgtgcaatgtaacatcagagattttgagacacaacgtggctttgttgaataaatcgaacttttgctgagttgaaggatcagatcacgcatcttcccgacaacgcagaccgttccgtggcaaagcaaaagttcaaaatcaccaactggtcgcgatccggtgtatgc

SEQ ID NO: 167 - DNA, 58 bp, Artificial Sequence
  primer
gcacttaccttaactggtaggtgcttttttcaattctgattagaaaaactcatcgagc

SEQ ID NO: 168 - DNA, 18 bp, Artificial Sequence
  primer
ggtacccggggatcatgc

SEQ ID NO: 169 - DNA, 35 bp, Artificial Sequence
  primer
ccaagcttgcatgccggtaggtggcgtatcagact

SEQ ID NO: 170 - DNA, 35 bp, Artificial Sequence
  primer
acgcgagaaacggcactagttgagggcctctaaat

SEQ ID NO: 171 - DNA, 35 bp, Artificial Sequence
  primer
gagtgttcgttaaaaatggcacaggttatggactt

SEQ ID NO: 172 - DNA, 35 bp, Artificial Sequence
  primer
cggtacccggggatcttagtagcggtagtgctccg

SEQ ID NO: 173 - DNA, 35 bp, Artificial Sequence
  primer
gaggccctcaactagtgccgtttctcgcgttgtgt

SEQ ID NO: 174 - DNA, 35 bp, Artificial Sequence
  primer
cataacctgtgccatttttaacgaacactcctcgc

SEQ ID NO: 175 - DNA, 1437 bp, Corynebacterium glutamicum
atggcacaggttatggacttcaaggttgccgatctttcactagcagaggcaggacgtcaccagattcgtcttgcagagtatgagatgccaggtctcatgcagttgcgcaaggaattcgcagacgagcagcctttgaagggcgcccgaattgctggttccatccacatgacggtccagaccgccgtgcttattgagaccctcactgctttgggcgctgaggttcgttgggcttcctgcaacattttctccacccaggatgaggctgcagcggctatcgttgtcggctccggcaccgtcgaagagccagctggtgttccagtattcgcgtggaagggtgagtcactggaggagtactggtggtgcatcaaccagatcttcagctggggcgatgagctgccaaacatgatcctcgacgacggcggtgacgccaccatggctgttattcgcggtcgcgaatacgagcaggctggtctggttccaccagcagaggccaacgattccgatgagtacatcgcattcttgggcatgctgcgtgaggttcttgctgcagagcctggcaagtggggcaagatcgctgaggccgttaagggtgtcaccgaggaaaccaccaccggtgtgcaccgcctgtaccacttcgctgaagaaggcgtactgcctttcccagcgatgaacgtcaacgacgctgtcaccaagtccaagtttgataacaagtacggcacccgccactccctgatcgacggcatcaaccgcgccaccgacatgctcatgggcggcaagaacgtgcttgtctgcggttacggtgatgtcggcaagggctgcgctgaggctttcgacggccagggcgctcgcgtcaaggtcaccgaagctgacccaatcaacgctcttcaggctctgatggatggctactctgtggtcaccgttgatgaggccatcgaggacgccgacatcgtgatcaccgcgaccggtaacaaggacatcatttccttcgagcagatgctcaagatgaaggatcacgctctgctgggcaacatcggtcactttgataatgagatcgatatgcattccctgttgcaccgcgacgacgtcacccgcaccacgatcaagccacaggtcgacgagttcaccttctccaccggtcgctccatcatcgtgctgtctgaaggccgtctgctaaaccttggcaacgccaccggacacccatcatttgtcatgtccaactctttcgccgatcagaccattgcgcagatcgaactgttccaaaacgaaggacagtacgagaacgaggtctaccgtctgcctaaggttctcgacgaaaaggtggcacgcatccacgttgaggctctcggcggtcagctcaccgaactgaccaaggagcaggctgagtacatcggcgttgacgttgcaggtccattcaagccggagcactaccgctactaa

SEQ ID NO: 176 - protein, 478 aa, Corynebacterium glutamicum
MAQVMDFKVADLSLAEAGRHQIRLAEYEMPGLMQLRKEFADEQPLKGARIAGSIHMTVQTAVLIETLTALGAEVRWASCNIFSTQDEAAAAIVVGSGTVEEPAGVPVFAWKGESLEEYWWCINQIFSWGDELPNMILDDGGDATMAVIRGREYEQAGLVPPAEANDSDEYIAFLGMLREVLAAEPGKWGKIAEAVKGVTEETTTGVHRLYHFAEEGVLPFPAMNVNDAVTKSKFDNKYGTRHSLIDGINRATDMLMGGKNVLVCGYGDVGKGCAEAFDGQGARVKVTEADPINALQALMDGYSVVTVDEAIEDADIVITATGNKDIISFEQMLKMKDHALLGNIGHFDNEIDMHSLLHRDDVTRTTIKPQVDEFTFSTGRSIIVLSEGRLLNLGNATGHPSFVMSNSFADQTIAQIELFQNEGQYENEVYRLPKVLDEKVARIHVEALGGQLTELTKEQAEYIGVDVAGPFKPEHYRY

SEQ ID NO: 177 - DNA, 1563 bp, Corynebacterium glutamicum
atgagcgatgatcgtaaggcaattaaacgcgcactaattagcgtgtatgacaagactggcctggaggatctagcccaggcacttcaccgcgcgaacgtggaaattgtttccaccggatccactgcggcgaagattgctgagcttggtattcctgttaccccggttgaggagctcaccggtttccctgagtgccttgagggccgtgtgaagacactgcatcctaaggttcacgctggcatcttggcggacacccgcaaggaagaccacctgcgtcagctcaaggaacttgaggtcgccccattccagcttgtcgtggtgaacctgtacccatttgctgagaccgttgcgtccggcgccgatttcgatgcttgcgttgagcagatcgacatcggaggcccatccatggttcgtgctgcggcaaagaaccacccatctgtcgctgtggttgtttcaccaaaccgctacgaggatgtccaggaagctttgaagaccggtggattctcccgcgcggagcgcaccaagttggctgctgaggctttccgccacaccgcaacctacgatgtcaccgttgcaacctggatgagcgagcagctggctgccgaagattctgagactgagttcccaggttggatcggcaccaccaacaccttgtcccgcagcttgcgttacggtgagaaccctcaccagtctgcagctttgtacgtgggcaacacccgcggacttgcacaggctaagcagttccacggcaaggaaatgagctacaacaactacaccgattctgatgctgcatggcgtgcagcgtgggatcacgagcgtccttgtgtagctatcatcaagcatgcaaacccttgtggcattgctgtttctgatgagtccatcgcagcggcacaccgcgaggcacacgcatgtgactctgtgtccgcattcggtggcgtcatcgcgtccaaccgtgaagtcagcgttgagatggctaaccaggttgcagagatcttcactgaggtcatcatcgctccttcctacgaagagggcgctgtggagatcctgagccagaagaagaacatccgtattcttcaggctgaagcacctgtgcgtaagggctttgagtcccgtgagatctccggcggtctgcttgttcaggaacgcgacttgatccacgctgagggcgacaactccgcaaactggactcttgctgccggctctgctgtttctcctgaggttctgaaggacctggagttcgcgtggactgcagttcgttccgtgaagtccaacgcaattctgttggctaagaacggcgctaccgttggcgttggcatgggacaggtcaaccgcgttgactctgctcgcttggctgtcgaccgtgcaggtgcagagcgcgctaccggttccgttgctgcttccgatgcgttcttcccattcgctgatggctttgaggttctcgctgaggctggcatcactgctgttgtgcagcctggtggatccattcgcgacaacgaggtcattgaggcagccaacaaggctggcgtgaccatgtacctgactggtgcgcgacacttcgctcactaa

SEQ ID NO: 178 - protein, 520 aa, Corynebacterium glutamicum
MSDDRKAIKRALISVYDKTGLEDLAQALHRANVEIVSTGSTAAKIAELGIPVTPVEELTGFPECLEGRVKTLHPKVHAGILADTRKEDHLRQLKELEVAPFQLVVVNLYPFAETVASGADFDACVEQIDIGGPSMVRAAAKNHPSVAVVVSPNRYEDVQEALKTGGFSRAERTKLAAEAFRHTATYDVTVATWMSEQLAAEDSETEFPGWIGTTNTLSRSLRYGENPHQSAALYVGNTRGLAQAKQFHGKEMSYNNYTDSDAAWRAAWDHERPCVAIIKHANPCGIAVSDESIAAAHREAHACDSVSAFGGVIASNREVSVEMANQVAEIFTEVIIAPSYEEGAVEILSQKKNIRILQAEAPVRKGFESREISGGLLVQERDLIHAEGDNSANWTLAAGSAVSPEVLKDLEFAWTAVRSVKSNAILLAKNGATVGVGMGQVNRVDSARLAVDRAGAERATGSVAASDAFFPFADGFEVLAEAGITAVVQPGGSIRDNEVIEAANKAGVTMYLTGARHFAH

SEQ ID NO: 179 - DNA, 1563 bp, Corynebacterium glutamicum
atgagcgatgatcgtaaggcaattaaacgcgcactaattagcgtgtatgacaagactggcctggaggatctagcccaggcacttcaccgcgcgaacgtggaaattgttttcaccggatccactgcggcgaagattgctgagcttggtattcctgttaccccggttgaggagctcaccggtttccctgagtgccttgagggccgtgtgaagacactgcatcctaaggttcacgctggcatcttggcggacacccgcaaggaagaccacctgcgtcagctcaaggaacttgaggtcgccccattccagcttgtcgtggtgaacctgtacccatttgctgagaccgttgcgtccggcgccgatttcgatgcttgcgttgagcagatcgacatcggaggcccatccatggttcgtgctgcggcaaagaaccacccatctgtcgctgtggttgtttcaccaaaccgctacgaggatgtccaggaagctttgaagaccggtggattctcccgcgcggagcgcaccaagttggctgctgaggctttccgccacaccgcaacctacgatgtcaccgttgcaacctggatgagcgagcagctggctgccgaagattctgagactgagttcccaggttggatcggcaccaccaacaccttgtcccgcagcttgcgttacggtgagaaccctcaccagtctgcagctttgtacgtgggcaacacccgcggacttgcacaggctaagcagttccacggcaaggaaatgagctacaacaactacaccgattctgatgctgcatggcgtgcagcgtgggatcacgagcgtccttgtgtagctatcatcaagcatgcaaacccttgtggcattgctgtttctgatgagtccatcgcagcggcacaccgcgaggcacacgcatgtgactctgtgtccgcattcggtggcgtcatcgcgtccaaccgtgaagtcagcgttgagatggctaaccaggttgcagagatcttcactgaggtcatcatcgctccttcctacgaagagggcgctgtggagatcctgagccagaagaagaacatccgtattcttcaggctgaagcacctgtgcgtaagggctttgagtcccgtgagatctccggcggtctgcttgttcaggaacgcgacttgatccacgctgagggcgacaactccgcaaactggactcttgctgccggctctgctgtttctcctgaggttctgaaggacctggagttcgcgtggactgcagttcgttccgtgaagtccaacgcaattctgttggctaagaacggcgctaccgttggcgttggcatgggacaggtcaaccgcgttgactctgctcgcttggctgtcgaccgtgcaggtgcagagcgcgctaccggttccgttgctgcttccgatgcgttcttcccattcgctgatggctttgaggttctcgctgaggctggcatcactgctgttgtgcagcctggtggatccattcgcgacaacgaggtcattgaggcagccaacaaggctggcgtgaccatgtacctgactggtgcgcgacacttcgctcactaa

SEQ ID NO: 180 - protein, 520 aa, Corynebacterium glutamicum
MSDDRKAIKRALISVYDKTGLEDLAQALHRANVEIVFTGSTAAKIAELGIPVTPVEELTGFPECLEGRVKTLHPKVHAGILADTRKEDHLRQLKELEVAPFQLVVVNLYPFAETVASGADFDACVEQIDIGGPSMVRAAAKNHPSVAVVVSPNRYEDVQEALKTGGFSRAERTKLAAEAFRHTATYDVTVATWMSEQLAAEDSETEFPGWIGTTNTLSRSLRYGENPHQSAALYVGNTRGLAQAKQFHGKEMSYNNYTDSDAAWRAAWDHERPCVAIIKHANPCGIAVSDESIAAAHREAHACDSVSAFGGVIASNREVSVEMANQVAEIFTEVIIAPSYEEGAVEILSQKKNIRILQAEAPVRKGFESREISGGLLVQERDLIHAEGDNSANWTLAAGSAVSPEVLKDLEFAWTAVRSVKSNAILLAKNGATVGVGMGQVNRVDSARLAVDRAGAERATGSVAASDAFFPFADGFEVLAEAGITAVVQPGGSIRDNEVIEAANKAGVTMYLTGARHFAH

SEQ ID NO: 181 - DNA, 36 bp, Artificial Sequence
  primer
cggtacccggggatcctcaacctcctggcgtcagtt

SEQ ID NO: 182 - DNA, 35 bp, Artificial Sequence
  primer
acaatgagtttacgctcaacctgcttgattctttc

SEQ ID NO: 183 - DNA, 35 bp, Artificial Sequence
  primer
attccagcttgtcgtggtgaacctgtacccatttg

SEQ ID NO: 184 - DNA, 36 bp, Artificial Sequence
  primer
ccaagcttgcatgccgatcaagtcgcgttcctgaac

SEQ ID NO: 185 - DNA, 400 bp, Artificial Sequence
  primer
gcgtaaactcattgtagaagtcctgaacagcgtggaattttcgcgtcagggtggcgtacaactcaactggagaggctaaatccttcatgagcgatgatcgtaaggcaattaaacgcgcactaattagcgtgtatgacaagactggcctggaggatctagcccaggcacttcaccgcgcgaacgtggaaattgttttcaccggatccactgcggcgaagattgctgagcttggtattcctgttaccccggttgaggagctcaccggtttccctgagtgccttgagggccgtgtgaagacactgcatcctaaggttcacgctggcatcttggcggacacccgcaaggaagaccacctgcgtcagctcaaggaacttgaggtcgccccattccagcttgtcgt

SEQ ID NO: 186 - DNA, 20 bp, Artificial Sequence
  primer
cagcactgtgtttcctcgtc

SEQ ID NO: 187 - DNA, 20 bp, Artificial Sequence
  primer
caggtccttcagaacctcag